European Patent Application EP 4 241 785 A2, published September 13, 2023. Title: INFLUENZA VIRUS VACCINES AND USES THEREOF. Applicant: ICAHN SCHOOL OF MEDICINE AT MOUNT SINAI. The sequence listing filed with the application follows.

SEQUENCE LISTING (582 sequences)

SEQ ID NO: 1 - protein, 565 aa, Influenza virus A
  source 1..565: note = influenza virus A hemagglutinin subtype H1
MKANLLVLLCALAAADADTICIGYHANNSTDTVDTVLEKNVTVTHSVNLLEDSHNGKLCRLKGIAPLQLGKCNIAGWLLGNPECDPLLPVRSWSYIVETPNSENGICYPGDFIDYEELREQLSSVSSFERFEIFPKESSWPNHNTNGVTAACSHEGKSSFYRNLLWLTEKEGSYPKLKNSYVNKKGKEVLVLWGIHHPPNSKEQQNLYQNENAYVSVVTSNYNRRFTPEIAERPKVRDQAGRMNYYWTLLKPGDTIIFEANGNLIAPMYAFALSRGFGSGIITSNASMHECNTKCQTPLGAINSSLPYQNIHPVTIGECPKYVRSAKLRMVTGLRNNPSIQSRGLFGAIAGFIEGGWTGMIDGWYGYHHQNEQGSGYAADQKSTQNAINGITNKVNTVIEKMNIQFTAVGKEFNKLEKRMENLNKKVDDGFLDIWTYNAELLVLLENERTLDFHDSNVKNLYEKVKSQLKNNAKEIGNGCFEFYHKCDNECMESVRNGTYDYPKYSEESKLNREKVDGVKLESMGIYQILAIYSTVASSLVLLVSLGAISFWMCSNGSLQCRICI

SEQ ID NO: 2 - protein, 562 aa, Influenza virus A
  source 1..562: note = influenza virus A hemagglutinin subtype H2
MAIIYLILLFTAVRGDQICIGYHSNNSTEKVDTILERNVTVTHAQNILEKTHNGKLCKLNGIPPLELGDCSIAGWLLGNPECDRLLTVPEWSYIMEKENPRNGLCYPGSFNDYEELKHLLSSVTHFEKVKILPKDRWTQHTTTGGSRACAVSGNPSFFRNMVWLTKKGSNYPIAKGSYNNTSGEQMLIIWGVHHPNDETEQRTLYQNVGTYVSIGTSTLNKRSIPVIATRPKVNGQGGRMEFSWTILDIWDTINFESTGNLIAPEYGFRISKRGSSGIMKTEGTLENCETKCQTPLGAINTTLPFHNVHPLTIGECPKYVKSERLVLATGLRNVPQIESRGLFGAIAGFIEGGWQGMIDGWYGYHHSNDQGSGYAADKESTQKAIDGITNRVNSVIEKMNTQFEAVGKEFSNLEKRLENLNKKMEDGFLDVWTYNAELLVLMENERTLDFHDSNVKNLYDRVRMQLRDNAKELGNGCFEFYHKCDDECMNSVKNGTYDYPKYEEESKLNRNEIKGVKLSNMGVYQILAIYATVAGSLSLAIMIAGISLWMCSNGSLQCRICI

SEQ ID NO: 3 - protein, 566 aa, Influenza virus A
  source 1..566: note = influenza virus A hemagglutinin subtype H3
MKTIIALSYIFCLALGQDLPGNDNSTATLCLGHHAVPNGTLVKTITDDQIEVTNATELVQSSSTGKICNNPHRILDGIDCTLIDALLGDPHCDVFQNETWDLFVERSKAFSNCYPYDVPDYASLRSLVASSGTLEFITEGFTWTGVTQNGGSNACKRGPGNGFFSRLNWLTKSGSTYPVLNVTMPNNDNFDKLYIWGVHHPSTNQEQTSLYVQESGRVTVSTRRSQQSIIPNIGSRPWVRGQSSRISIYWTIVKPGDVLVINSNGNLIAPRGYFKMRTGKSSIMSSDAPIDTCISECITPNGSIPNDKPFQNVNKITYGACPKYVKQNTLKLATGMRNVPEKQTRGLFGAIAGFIENGWEGMIDGWYGFRHQNSEGTGQAADLKSTQAAIDQINGKLNRVIEKTNEKFHQIEKEFSEVEGRIQDLEKYVEDTKIDLWSYNAELLVALENQHTIDLTDSEMNKLFEKTRRQLRENAEDMGNGCFKIYHKCDNACIESIRNGTYDHDVYRDEALNNRFQIKGVELKSGYKDWILWISFAISCFLLCVVLLGFIMWACQRGNIRCNICI

SEQ ID NO: 4 - protein, 564 aa, Influenza virus A
  source 1..564: note = influenza virus A hemagglutinin subtype H4
MLSIVILFLLIAENSSQNYTGNPVICMGHHAVANGTMVKTLADDQVEVVTAQELVESQNLPELCPSPLRLVDGQTCDIINGALGSPGCDHLNGAEWDVFIERPNAVDTCYPFDVPEYQSLRSILANNGKFEFIAEEFQWNTVKQNGKSGACKRANVDDFFNRLNWLVKSDGNAYPLQNLTKINNGDYARLYIWGVHHPSTSTEQTNLYKNNPGRVTVSTKTSQTSVVPDIGSRPLVRGQSGRVSFYWTIVEPGDLIVFNTIGNLIAPRGHYKLNNQKKSTILNTAIPIGSCVSKCHTDKGSLSTTKPFQNISRIAVGDCPRYVKQGSLKLATGMRNIPEKASRGLFGAIAGFIENGWQGLIDGWYGFRHQNAEGTGTAADLKSTQAAIDQINGKLNRLIEKTNDKYHQIEKEFEQVEGRIQDLENYVEDTKIDLWSYNAELLVALENQHTIDVTDSEMNKLFERVRRQLRENAEDKGNGCFEIFHKCDNNCIESIRNGTYDHDIYRDEAINNRFQIQGVKLTQGYKDIILWISFSISCFLLVALLLAFILWACQNGNIRCQICI

SEQ ID NO: 5 - protein, 564 aa, Influenza virus A
  source 1..564: note = influenza virus A hemagglutinin subtype H5
MERIVLLLAIVSLVKSDQICIGYHANKSTKQVDTIMEKNVTVTHAQDILERTHNGKLCSLNGVKPLILRDCSVAGWLLGNPMCDEFLNLPEWLYIVEKDNPINSLCYPGDFNDYEELKYLLSSTNHFEKIRIIPRSSWSNHDASSGVSSACPYIGRSSFLRNVVWLIKKNNTYPTIKRSYNNTNQEDLLILWGIHHPNDAAEQTKLYQNPTTYVSVGTSTLNQRSIPEIATRPKVNGQSGRMEFFWTILKPNDAINFESNGNFIAPRYAYKIVKKGDSAIMKSGLAYGNCDTKCQTPVGEINSSMPFHNIHPHTIGECPKYVKSDRLVLATGLRNVPQRKKRGLFGAIAGFIEGGWQGMVDGWYGYHHSNEQGSGYAADKESTQKAIDGITNKVNSIIDKMNTRFEAVGKEFNNLERRVENLNKKMEDGFLDVWTYNVELLVLMENERTLDFHDSNVNNLYDKVRLQLKDNARELGNGCFEFYHKCDNECMESVRNGTYDYPQYSEEARLNREEISGVKLESMGVYQILSIYSTVASSLALAIMIAGLSFWMCSNGSLQCRICI

SEQ ID NO: 6 - protein, 566 aa, Influenza virus A
  source 1..566: note = influenza virus A hemagglutinin subtype H6
MIAIIVVAILATAGRSDKICIGYHANNSTTQIDTILEKNVTVTHSVELLENQKEERFCKILKKAPLDLKGCTIEGWILGNPQCDLLLGDQSWSYIVERPTAQNGICYPGVLNEVEELKALIGSGERVERFEMFPKSTWTGVDTSSGVTRACPYNSGSSFYRNLLWIIKTKSAAYSVIKGAYNNTGNQPILYFWGVHHPPDTNEQNTLYGSGDRYVRMGTESMNFAKSPEIAARPAVNGQRGRIDYYWSILKPGETLNVESNGNLIAPWYAFRFVSTSNKGAVFKSNLPIENCDATCQTVAGVLRTNKTFQNVSPLWIGECPKYVKSESLRLATGLRNVPQIETRGLFGAIAGFIEGGWTGMIDGWYGYHHENSQGSGYAADRESTQKAVDGITNKVNSIIDKMNTQFEAVDHEFSNLERRIDNLNKRMEDGFLDVWTYNAELLVLLENERTLDLHDANVKNLYERVKSQLRDNAMILGNGCFEFWHKCDDECMESVKNGTYDYPKYQDESKLNRQEIESVKLESLGVYQILAIYSTVSSSLVLVGLIIAVGLWMCSNGSMQCRICI

SEQ ID NO: 7 - protein, 563 aa, Influenza virus A
  source 1..563: note = influenza virus A hemagglutinin subtype H7
MNTQILVFALVAVIPTNADKICLGHHAVSNGTKVNTLTERGVEVVNATETVERTNIPKICSKGKRTTDLGQCGLLGTITGPPQCDQFLEFSADLIIERREGNDVCYPGKFVNEEALRQILRGSGGIDKETMGFTYSGIRTNGTTSACRRSGSSFYAEMEWLLSNTDNASFPQMTKSYKNTRRESALIVWGIHHSGSTTEQTKLYGSGNKLITVGSSKYHQSFVPSPGTRPQINGQSGRIDFHWLILDPNDTVTFSFNGAFIAPNRASFLRGKSMGIQSDVQVDANCEGECYHSGGTITSRLPFQNINSRAVGKCPRYVKQESLLLATGMKNVPEPSKKRKKRGLFGAIAGFIENGWEGLVDGWYGFRHQNAQGEGTAADYKSTQSAIDQITGKLNRLIEKTNQQFELIDNEFTEVEKQIGNLINWTKDSITEVWSYNAELIVAMENQHTIDLADSEMNRLYERVRKQLRENAEEDGTGCFEIFHKCDDDCMASIRNNTYDHSKYREEAMQNRIQIDPVKLSSGYKDVILWFSFGASCFLLLAIAMGLVFICVKNGNMRCTICI

SEQ ID NO: 8 - protein, 565 aa, Influenza virus A
  source 1..565: note = influenza virus A hemagglutinin subtype H8
MEKFIAIATLASTNAYDRICIGYQSNNSTDTVNTLIEQNVPVTQTMELVETEKHPAYCNTDLGAPLELRDCKIEAVIYGNPKCDIHLKDQGWSYIVERPSAPEGMCYPGSVENLEELRFVFSSAASYKRIRLFDYSRWNVTRSGTSKACNASTGGQSFYRSINWLTKKEPDTYDFNEGAYVNNEDGDIIFLWGIHHPPDTKEQTTLYKNANTLSSVTTNTINRSFQPNIGPRPLVRGQQGRMDYYWGILKRGETLKIRTNGNLIAPEFGYLLKGESYGRIIQNEDIPIGNCNTKCQTYAGAINSSKPFQNASRHYMGECPKYVKKASLRLAVGLRNTPSVEPRGLFGAIAGFIEGGWSGMIDGWYGFHHSNSEGTGMAADQKSTQEAIDKITNKVNNIVDKMNREFEVVNHEFSEVEKRINMINDKIDDQIEDLWAYNAELLVLLENQKTLDEHDSNVKNLFDEVKRRLSANAIDAGNGCFDILHKCDNECMETIKNGTYDHKEYEEEAKLERSKINGVKLEENTTYKILSIYSTVAASLCLAILIAGGLILGMQNGSCRCMFCI

SEQ ID NO: 9 - protein, 560 aa, Influenza virus A
  source 1..560: note = influenza virus A hemagglutinin subtype H9
METKAIIAALLMVTAANADKICIGYQSTNSTETVDTLTESNVPVTHTKELLHTEHNGMLCATDLGHPLILDTCTIEGLIYGNPSCDILLGGKEWSYIVERSSAVNGMCYPGNVENLEELRSLFSSAKSYKRIQIFPDKTWNVTYSGTSRACSNSFYRSMRWLTHKSNSYPFQNAHYTNNERENILFMWGIHHPPTDTEQTDLYKNADTTTSVTTEDINRTFKPVIGPRPLVNGQQGRIDYYWSVLKPGQTLRIRSNGNLIAPWYGHVLTGESHGRILKTDLNNGNCVVQCQTEKGGLNTTLPFHNISKYAFGNCPKYVGVKSLKLPVGLRNVPAVSSRGLFGAIAGFIEGGWPGLVAGWYGFQHSNDQGVGMAADKGSTQKAIDKITSKVNNIIDKMNKQYEVIDHEFNELEARLNMINNKIDDQIQDIWAYNAELLVLLENQKTLDEHDANVNNLYNKVKRALGSNAVEDGNGCFELYHKCDDQCMETIRNGTYDRQKYQEESRLERQKIEGVKLESEGTYKILTIYSTVASSLVLAMGFAAFLFWAMSNGSCRCNICI

SEQ ID NO: 10 - protein, 561 aa, Influenza virus A
  source 1..561: note = influenza virus A hemagglutinin subtype H10
MYKVVVIIALLGAVKGLDRICLGHHAVANGTIVKTLTNEQEEVTNATETVESTNLNKLCMKGRSYKDLGNCHPVGMLIGTPVCDPHLTGTWDTLIERENAIAHCYPGATINEEALRQKIMESGGISKMSTGFTYGSSITSAGTTKACMRNGGDSFYAELKWLVSKTKGQNFPQTTNTYRNTDTAEHLIIWGIHHPSSTQEKNDLYGTQSLSISVESSTYQNNFVPVVGARPQVNGQSGRIDFHWTLVQPGDNITFSDNGGLIAPSRVSKLTGRDLGIQSEALIDNSCESKCFWRGGSINTKLPFQNLSPRTVGQCPKYVNQRSLLLATGMRNVPEVVQGRGLFGAIAGFIENGWEGMVDGWYGFRHQNAQGTGQAADYKSTQAAIDQITGKLNRLIEKTNTEFESIESEFSETEHQIGNVINWTKDSITDIWTYNAELLVAMENQHTIDMADSEMLNLYERVRKQLRQNAEEDGKGCFEIYHTCDDSCMESIRNNTYDHSQYREEALLNRLNINPVKLSSGYKDIILWFSFGESCFVLLAVVMGLVFFCLKNGNMRCTICI

SEQ ID NO: 11 - protein, 565 aa, Influenza virus A
  source 1..565: note = influenza virus A hemagglutinin subtype H11
MEKTLLFAAIFLCVKADEICIGYLSNNSTDKVDTIIENNVTVTSSVELVETEHTGSFCSINGKQPISLGDCSFAGWILGNPMCDELIGKTSWSYIVEKPNPTNGICYPGTLESEEELRLKFSGVLEFNKFEVFTSNGWGAVNSGVGVTAACKFGGSNSFFRNMVWLIHQSGTYPVIKRTFNNTKGRDVLIVWGIHHPATLTEHQDLYKKDSSYVAVGSETYNRRFTPEINTRPRVNGQAGRMTFYWKIVKPGESITFESNGAFLAPRYAFEIVSVGNGKLFRSELNIESCSTKCQTEIGGINTNKSFHNVHRNTIGDCPKYVNVKSLKLATGPRNVPAIASRGLFGAIAGFIEGGWPGLINGWYGFQHRDEEGTGIAADKESTQKAIDQITSKVNNIVDRMNTNFESVQHEFSEIEERINQLSKHVDDSVVDIWSYNAQLLVLLENEKTLDLHDSNVRNLHEKVRRMLKDNAKDEGNGCFTFYHKCDNKCIERVRNGTYDHKEFEEESKINRQEIEGVKLDSSGNVYKILSIYSCIASSLVLAALIMGFMFWACSNGSCRCTICI

SEQ ID NO: 12 - protein, 564 aa, Influenza virus A
  source 1..564: note = influenza virus A hemagglutinin subtype H12
MEKFIILSTVLAASFAYDKICIGYQTNNSTETVNTLSEQNVPVTQVEELVHRGIDPILCGTELGSPLVLDDCSLEGLILGNPKCDLYLNGREWSYIVERPKEMEGVCYPGSIENQEELRSLFSSIKKYERVKMFDFTKWNVTYTGTSKACNNTSNQGSFYRSMRWLTLKSGQFPVQTDEYKNTRDSDIVFTWAIHHPPTSDEQVKLYKNPDTLSSVTTVEINRSFKPNIGPRPLVRGQQGRMDYYWAVLKPGQTVKIQTNGNLIAPEYGHLITGKSHGRILKNNLPMGQCVTECQLNEGVMNTSKPFQNTSKHYIGKCPKYIPSGSLKLAIGLRNVPQVQDRGLFGAIAGFIEGGWPGLVAGWYGFQHQNAEGTGIAADRDSTQRAIDNMQNKLNNVIDKMNKQFEVVNHEFSEVESRINMINSKIDDQITDIWAYNAELLVLLENQKTLDEHDANVRNLHDRVRRVLRENAIDTGDGCFEILHKCDNNCMDTIRNGTYNHKEYEEESKIERQKVNGVKLEENSTYKILSIYSSVASSLVLLLMIIGGFIFGCQNGNVRCTFCI

SEQ ID NO: 13 - protein, 566 aa, Influenza virus A
  source 1..566: note = influenza virus A hemagglutinin subtype H13
MALNVIATLTLISVCVHADRICVGYLSTNSSERVDTLLENGVPVTSSIDLIETNHTGTYCSLNGVSPVHLGDCSFEGWIVGNPACTSNFGIREWSYLIEDPAAPHGLCYPGELNNNGELRHLFSGIRSFSRTELIPPTSWGEVLDGTTSACRDNTGTNSFYRNLVWFIKKNTRYPVISKTYNNTTGRDVLVLWGIHHPVSVDETKTLYVNSDPYTLVSTKSWSEKYKLETGVRPGYNGQRSWMKIYWSLIHPGEMITFESNGGFLAPRYGYIIEEYGKGRIFQSRIRMSRCNTKCQTSVGGINTNRTFQNIDKNALGDCPKYIKSGQLKLATGLRNVPAISNRGLFGAIAGFIEGGWPGLINGWYGFQHQNEQGTGIAADKESTQKAIDQITTKINNIIDKMNGNYDSIRGEFNQVEKRINMLADRIDDAVTDIWSYNAKLLVLLENDKTLDMHDANVKNLHEQVRRELKDNAIDEGNGCFELLHKCNDSCMETIRNGTYDHTEYAEESKLKRQEIDGIKLKSEDNVYKALSIYSCIASSVVLVGLILSFIMWACSSGNCRFNVCI

SEQ ID NO: 14 - protein, 568 aa, Influenza virus A
  source 1..568: note = influenza virus A hemagglutinin subtype H14
MIALILVALALSHTAYSQITNGTTGNPIICLGHHAVENGTSVKTLTDNHVEVVSAKELVETNHTDELCPSPLKLVDGQDCHLINGALGSPGCDRLQDTTWDVFIERPTAVDTCYPFDVPDYQSLRSILASSGSLEFIAEQFTWNGVKVDGSSSACLRGGRNSFFSRLNWLTKATNGNYGPINVTKENTGSYVRLYLWGVHHPSSDNEQTDLYKVATGRVTVSTRSDQISIVPNIGSRPRVRNQSGRISIYWTLVNPGDSIIFNSIGNLIAPRGHYKISKSTKSTVLKSDKRIGSCTSPCLTDKGSIQSDKPFQNVSRIAIGNCPKYVKQGSLMLATGMRNIPGKQAKGLFGAIAGFIENGWQGLIDGWYGFRHQNAEGTGTAADLKSTQAAIDQINGKLNRLIEKTNEKYHQIEKEFEQVEGRIQDLEKYVEDTKIDLWSYNAELLVALENQHTIDVTDSEMNKLFERVRRQLRENAEDQGNGCFEIFHQCDNNCIESIRNGTYDHNIYRDEAINNRIKINPVTLTMGYKDIILWISFSMSCFVFVALILGFVLWACQNGNIRCQICI

SEQ ID NO: 15 - protein, 570 aa, Influenza virus A
  source 1..570: note = influenza virus A hemagglutinin subtype H15
MNTQIIVILVLGLSMVKSDKICLGHHAVANGTKVNTLTERGVEVVNATETVEITGIDKVCTKGKKAVDLGSCGILGTIIGPPQCDLHLEFKADLIIERRNSSDICYPGRFTNEEALRQIIRESGGIDKESMGFRYSGIRTDGATSACKRTVSSFYSEMKWLSSSMNNQVFPQLNQTYRNTRKEPALIVWGVHHSSSLDEQNKLYGTGNKLITVGSSKYQQSFSPSPGARPKVNGQAGRIDFHWMLLDPGDTVTFTFNGAFIAPDRATFLRSNAPSGIEYNGKSLGIQSDAQIDESCEGECFYSGGTINSPLPFQNIDSRAVGKCPRYVKQSSLPLALGMKNVPEKIRTRGLFGAIAGFIENGWEGLIDGWYGFRHQNAQGQGTAADYKSTQAAIDQITGKLNRLIEKTNKQFELIDNEFTEVEQQIGNVINWTRDSLTEIWSYNAELLVAMENQHTIDLADSEMNKLYERVRRQLRENAEEDGTGCFEIFHRCDDQCMESIRNNTYNHTEYRQEALQNRIMINPVKLSSGYKDVILWFSFGASCVMLLAIAMGLIFMCVKNGNLRCTICI

SEQ ID NO: 16 - protein, 565 aa, Influenza virus A
  source 1..565: note = influenza virus A hemagglutinin subtype H16
MMIKVLYFLIIVLGRYSKADKICIGYLSNNSSDTVDTLTENGVPVTSSVDLVETNHTGTYCSLNGISPIHLGDCSFEGWIVGNPSCATNINIREWSYLIEDPNAPNKFCYPGELDNNGELRHLFSGVNSFSRTELINPSKWGNVLDGVTASCLDRGASSFYRNLVWIVKKDEKYPVIKGDYNNTTGRDVLVLWGIHHPDTETTATNLYVNKNPYTLVSTKEWSKRYELEIGTRIGDGQRSWMKLYWHLMHPGERIMFESNGGLIAPRYGYIIEKYGTGRIFQSGVRMARCNTKCQTSLGGINTNKTFQNIERNALGDCPKYIKSGQLKLATGLRNVPSIGERGLFGAIAGFIEGGWPGLINGWYGFQHQNEQGTGIAADKASTQKAINEITTKINNIIEKMNGNYDSIRGEFNQVEKRINMLADRVDDAVTDIWSYNAKLLVLLENDRTLDLHDANVRNLHDQVKRALKSNAIDEGDGCFNLLHKCNDSCMETIRNGTYNHEDYREESQLKRQEIEGIKLKTEDNVYKVLSIYSCIASSIVLVGLILAFIMWACSNGSCRFNVCI

SEQ ID NO: 17 - protein, 342 aa, Influenza virus B
  source 1..342: note = influenza B virus hemagglutinin (in Fig. 3)
DRICTGITSSNSPHVVKTATQGEVNVTGVIPLTTTPTKSHFANLKGTQTRGKLCPNCLNCTDLDVALGRPKCMGTIPSAKASILHEVKPVTSGCFPIMHDRTKIRQLPNLLRGYENIRLSARNVTNAETAPGGPYIVGTSGSCPNVTNGNGFFATMAWAVPKNKTATNPLTVEVPYICTKGEDQITVWGFHSDDETQMVKLYGDSKPQKFTSSANGVTTHYVSQIGGFPNQAEDEGLPQSGRIVVDYMVQKPGKTGTIAYQRGVLLPQKVWCASGRSKVIKGSLPLIGEADCLHEKYGGLNKSKPYYTGEHAKAIGNCPIWVKTPLKLANGTKYRPPAKLLK

SEQ ID NO: 18 - protein, 17 aa, Influenza virus A
  source 1..17: note = influenza A HA subtype H1 signal peptides
MKANLLVLLCALAAADA

SEQ ID NO: 19 - protein, 15 aa, Influenza virus A
  source 1..15: note = influenza A HA subtype H2 signal peptides
MAIIYLILLFTAVRG

SEQ ID NO: 20 - protein, 16 aa, Influenza virus A
  source 1..16: note = influenza A HA subtype H3 signal peptides
MKTIIALSYIFCLALG

SEQ ID NO: 21 - protein, 16 aa, Influenza virus A
  source 1..16: note = influenza A HA subtype H4 signal peptides
MLSIVILFLLIAENSS

SEQ ID NO: 22 - protein, 16 aa, Influenza virus A
  source 1..16: note = influenza A HA subtype H5 signal peptides
MERIVLLLAIVSLVKS

SEQ ID NO: 23 - protein, 16 aa, Influenza virus A
  source 1..16: note = influenza A HA subtype H6 signal peptides
MIAIIVVAILATAGRS

SEQ ID NO: 24 - protein, 18 aa, Influenza virus A
  source 1..18: note = influenza A HA subtype H7 signal peptides
MNTQILVFALVAVIPTNA

SEQ ID NO: 25 - protein, 16 aa, Influenza virus A
  source 1..16: note = influenza A HA subtype H8 signal peptides
MEKFIAIATLASTNAY

SEQ ID NO: 26 - protein, 18 aa, Influenza virus A
  source 1..18: note = influenza A HA subtype H9 signal peptides
METKAIIAALLMVTAANA

SEQ ID NO: 27 - protein, 16 aa, Influenza virus A
  source 1..16: note = influenza A HA subtype H10 signal peptides
MYKVVVIIALLGAVKG

SEQ ID NO: 28 - protein, 16 aa, Influenza virus A
  source 1..16: note = influenza A HA subtype H11 signal peptides
MEKTLLFAAIFLCVKA

SEQ ID NO: 29 - protein, 17 aa, Influenza virus A
  source 1..17: note = influenza A HA subtype H12 signal peptides
MEKFIILSTVLAASFAY

SEQ ID NO: 30 - protein, 18 aa, Influenza virus A
  source 1..18: note = influenza A HA subtype H13 signal peptides
MALNVIATLTLISVCVHA

SEQ ID NO: 31 - protein, 17 aa, Influenza virus A
  source 1..17: note = influenza A HA subtype H14 signal peptides
MIALILVALALSHTAYS

SEQ ID NO: 32 - protein, 18 aa, Influenza virus A
  source 1..18: note = influenza A HA subtype H15 signal peptides
MNTQIIVILVLGLSMVKS

SEQ ID NO: 33 - protein, 19 aa, Influenza virus A
  source 1..19: note = influenza A HA subtype H16 signal peptides
MMIKVLYFLIIVLGRYSKA

SEQ ID NO: 34 - protein, 42 aa, Influenza virus A
  source 1..42: note = influenza A HA subtype H1 N-terminal stem segment
DTICIGYHANNSTDTVDTVLEKNVTVTHSVNLLEDSHNGKLC

SEQ ID NO: 35 - protein, 42 aa, Influenza virus A
  source 1..42: note = influenza A HA subtype H2 N-terminal stem segment
DQICIGYHSNNSTEKVDTILERNVTVTHAQNILEKTHNGKLC

SEQ ID NO: 36 - protein, 52 aa, Influenza virus A
  source 1..52: note = influenza A HA subtype H3 N-terminal stem segment
QDLPGNDNSTATLCLGHHAVPNGTLVKTITDDQIEVTNATELVQSSSTGKIC

SEQ ID NO: 37 - protein, 48 aa, Influenza virus A
  source 1..48: note = influenza A HA subtype H4 N-terminal stem segment
QNYTGNPVICMGHHAVANGTMVKTLADDQVEVVTAQELVESQNLPELC

SEQ ID NO: 38 - protein, 42 aa, Influenza virus A
  source 1..42: note = influenza A HA subtype H5 N-terminal stem segment
DQICIGYHANKSTKQVDTIMEKNVTVTHAQDILERTHNGKLC

SEQ ID NO: 39 - protein, 42 aa, Influenza virus A
  source 1..42: note = influenza A HA subtype H6 N-terminal stem segment
DKICIGYHANNSTTQIDTILEKNVTVTHSVELLENQKEERFC

SEQ ID NO: 40 - protein, 42 aa, Influenza virus A
  source 1..42: note = influenza A HA subtype H7 N-terminal stem segment
DKICLGHHAVSNGTKVNTLTERGVEVVNATETVERTNIPKIC

SEQ ID NO: 41 - protein, 42 aa, Influenza virus A
  source 1..42: note = influenza A HA subtype H8 N-terminal stem segment
DRICIGYQSNNSTDTVNTLIEQNVPVTQTMELVETEKHPAYC

SEQ ID NO: 42 - protein, 42 aa, Influenza virus A
  source 1..42: note = influenza A HA subtype H9 N-terminal stem segment
DKICIGYQSTNSTETVDTLTESNVPVTHTKELLHTEHNGMLC

SEQ ID NO: 43 - protein, 43 aa, Influenza virus A
  source 1..43: note = influenza A HA subtype H10 N-terminal stem segment
LDRICLGHHAVANGTIVKTLTNEQEEVTNATETVESTNLNKLC

SEQ ID NO: 44 - protein, 42 aa, Influenza virus A
  source 1..42: note = influenza A HA subtype H11 N-terminal stem segment
DEICIGYLSNNSTDKVDTIIENNVTVTSSVELVETEHTGSFC

SEQ ID NO: 45 - protein, 42 aa, Influenza virus A
  source 1..42: note = influenza A HA subtype H12 N-terminal stem segment
DKICIGYQTNNSTETVNTLSEQNVPVTQVEELVHRGIDPILC

SEQ ID NO: 46 - protein, 42 aa, Influenza virus A
  source 1..42: note = influenza A HA subtype H13 N-terminal stem segment
DRICVGYLSTNSSERVDTLLENGVPVTSSIDLIETNHTGTYC

SEQ ID NO: 47 - protein, 51 aa, Influenza virus A
  source 1..51: note = influenza A HA subtype H14 N-terminal stem segment
QITNGTTGNPIICLGHHAVENGTSVKTLTDNHVEVVSAKELVETNHTDELC

SEQ ID NO: 48 - protein, 42 aa, Influenza virus A
  source 1..42: note = influenza A HA subtype H15 N-terminal stem segment
DKICLGHHAVANGTKVNTLTERGVEVVNATETVEITGIDKVC

SEQ ID NO: 49 - protein, 42 aa, Influenza virus A
  source 1..42: note = influenza A HA subtype H16 N-terminal stem segment
DKICIGYLSNNSSDTVDTLTENGVPVTSSVDLVETNHTGTYC

SEQ ID NO: 50 - protein, 53 aa, Influenza virus A
  source 1..53: note = influenza A HA subtype H1 C-terminal stem segment
CNTKCQTPLGAINSSLPYQNIHPVTIGECPKYVRSAKLRMVTGLRNNPSIQSR

SEQ ID NO: 51 - protein, 53 aa, Influenza virus A
  source 1..53: note = influenza A HA subtype H2 C-terminal stem segment
CETKCQTPLGAINTTLPFHNVHPLTIGECPKYVKSERLVLATGLRNVPQIESR

SEQ ID NO: 52 - protein, 53 aa, Influenza virus A
  source 1..53: note = influenza A HA subtype H3 C-terminal stem segment
CISECITPNGSIPNDKPFQNVNKITYGACPKYVKQNTLKLATGMRNVPEKQTR

SEQ ID NO: 53 - protein, 53 aa, Influenza virus A
  source 1..53: note = influenza A HA subtype H4 C-terminal stem segment
CVSKCHTDKGSLSTTKPFQNISRIAVGDCPRYVKQGSLKLATGMRNIPEKASR

SEQ ID NO: 54 - protein, 53 aa, Influenza virus A
  source 1..53: note = influenza A HA subtype H5 C-terminal stem segment
CDTKCQTPVGEINSSMPFHNIHPHTIGECPKYVKSDRLVLATGLRNVPQRKKR

SEQ ID NO: 55 - protein, 53 aa, Influenza virus A
  source 1..53: note = influenza A HA subtype H6 C-terminal stem segment
CDATCQTVAGVLRTNKTFQNVSPLWIGECPKYVKSESLRLATGLRNVPQIETR

SEQ ID NO: 56 - protein, 57 aa, Influenza virus A
  source 1..57: note = influenza A HA subtype H7 C-terminal stem segment
CEGECYHSGGTITSRLPFQNINSRAVGKCPRYVKQESLLLATGMKNVPEPSKKRKKR

SEQ ID NO: 57 - protein, 53 aa, Influenza virus A
  source 1..53: note = influenza A HA subtype H8 C-terminal stem segment
CNTKCQTYAGAINSSKPFQNASRHYMGECPKYVKKASLRLAVGLRNTPSVEPR

SEQ ID NO: 58 - protein, 53 aa, Influenza virus A
  source 1..53: note = influenza A HA subtype H9 C-terminal stem segment
CVVQCQTEKGGLNTTLPFHNISKYAFGNCPKYVGVKSLKLPVGLRNVPAVSSR

SEQ ID NO: 59 - protein, 54 aa, Influenza virus A
  source 1..54: note = influenza A HA subtype H10 C-terminal stem segment
CESKCFWRGGSINTKLPFQNLSPRTVGQCPKYVNQRSLLLATGMRNVPEVVQGR

SEQ ID NO: 60 - protein, 53 aa, Influenza virus A
  source 1..53: note = influenza A HA subtype H11 C-terminal stem segment
CSTKCQTEIGGINTNKSFHNVHRNTIGDCPKYVNVKSLKLATGPRNVPAIASR

SEQ ID NO: 61 - protein, 53 aa, Influenza virus A
  source 1..53: note = influenza A HA subtype H12 C-terminal stem segment
CVTECQLNEGVMNTSKPFQNTSKHYIGKCPKYIPSGSLKLAIGLRNVPQVQDR

SEQ ID NO: 62 - protein, 53 aa, Influenza virus A
  source 1..53: note = influenza A HA subtype H13 C-terminal stem segment
CNTKCQTSVGGINTNRTFQNIDKNALGDCPKYIKSGQLKLATGLRNVPAISNR

SEQ ID NO: 63 - protein, 53 aa, Influenza virus A
  source 1..53: note = influenza A HA subtype H14 C-terminal stem segment
CTSPCLTDKGSIQSDKPFQNVSRIAIGNCPKYVKQGSLMLATGMRNIPGKQAK

SEQ ID NO: 64 - protein, 54 aa, Influenza virus A
  source 1..54: note = influenza A HA subtype H15 C-terminal stem segment
CEGECFYSGGTINSPLPFQNIDSRAVGKCPRYVKQSSLPLALGMKNVPEKIRTR

SEQ ID NO: 65 - protein, 53 aa, Influenza virus A
  source 1..53: note = influenza A HA subtype H16 C-terminal stem segment
CNTKCQTSLGGINTNKTFQNIERNALGDCPKYIKSGQLKLATGLRNVPSIGER

SEQ ID NO: 66 - protein, 222 aa, Influenza virus A
  source 1..222: note = influenza A HA subtype H1 HA2 domain
GLFGAIAGFIEGGWTGMIDGWYGYHHQNEQGSGYAADQKSTQNAINGITNKVNTVIEKMNIQFTAVGKEFNKLEKRMENLNKKVDDGFLDIWTYNAELLVLLENERTLDFHDSNVKNLYEKVKSQLKNNAKEIGNGCFEFYHKCDNECMESVRNGTYDYPKYSEESKLNREKVDGVKLESMGIYQILAIYSTVASSLVLLVSLGAISFWMCSNGSLQCRICI

SEQ ID NO: 67 - protein, 222 aa, Influenza virus A
  source 1..222: note = influenza A HA subtype H2 HA2 domain
GLFGAIAGFIEGGWQGMIDGWYGYHHSNDQGSGYAADKESTQKAIDGITNRVNSVIEKMNTQFEAVGKEFSNLEKRLENLNKKMEDGFLDVWTYNAELLVLMENERTLDFHDSNVKNLYDRVRMQLRDNAKELGNGCFEFYHKCDDECMNSVKNGTYDYPKYEEESKLNRNEIKGVKLSNMGVYQILAIYATVAGSLSLAIMIAGISLWMCSNGSLQCRICI

SEQ ID NO: 68 - protein, 221 aa, Influenza virus A
  source 1..221: note = influenza A HA subtype H3 HA2 domain
GLFGAIAGFIENGWEGMIDGWYGFRHQNSEGTGQAADLKSTQAAIDQINGKLNRVIEKTNEKFHQIEKEFSEVEGRIQDLEKYVEDTKIDLWSYNAELLVALENQHTIDLTDSEMNKLFEKTRRQLRENAEDMGNGCFKIYHKCDNACIESIRNGTYDHDVYRDEALNNRFQIKGVELKSGYKDWILWISFAISCFLLCVVLLGFIMWACQRGNIRCNICI

SEQ ID NO: 69 - protein, 221 aa, Influenza virus A
  source 1..221: note = influenza A HA subtype H4 HA2 domain
GLFGAIAGFIENGWQGLIDGWYGFRHQNAEGTGTAADLKSTQAAIDQINGKLNRLIEKTNDKYHQIEKEFEQVEGRIQDLENYVEDTKIDLWSYNAELLVALENQHTIDVTDSEMNKLFERVRRQLRENAEDKGNGCFEIFHKCDNNCIESIRNGTYDHDIYRDEAINNRFQIQGVKLTQGYKDIILWISFSISCFLLVALLLAFILWACQNGNIRCQICI

SEQ ID NO: 70 - protein, 222 aa, Influenza virus A
  source 1..222: note = influenza A HA subtype H5 HA2 domain
GLFGAIAGFIEGGWQGMVDGWYGYHHSNEQGSGYAADKESTQKAIDGITNKVNSIIDKMNTRFEAVGKEFNNLERRVENLNKKMEDGFLDVWTYNVELLVLMENERTLDFHDSNVNNLYDKVRLQLKDNARELGNGCFEFYHKCDNECMESVRNGTYDYPQYSEEARLNREEISGVKLESMGVYQILSIYSTVASSLALAIMIAGLSFWMCSNGSLQCRICI

SEQ ID NO: 71 - protein, 222 aa, Influenza virus A
  source 1..222: note = influenza A HA subtype H6 HA2 domain
GLFGAIAGFIEGGWTGMIDGWYGYHHENSQGSGYAADRESTQKAVDGITNKVNSIIDKMNTQFEAVDHEFSNLERRIDNLNKRMEDGFLDVWTYNAELLVLLENERTLDLHDANVKNLYERVKSQLRDNAMILGNGCFEFWHKCDDECMESVKNGTYDYPKYQDESKLNRQEIESVKLESLGVYQILAIYSTVSSSLVLVGLIIAVGLWMCSNGSMQCRICI

SEQ ID NO: 72 - protein, 221 aa, Influenza virus A
  source 1..221: note = influenza A HA subtype H7 HA2 domain
GLFGAIAGFIENGWEGLVDGWYGFRHQNAQGEGTAADYKSTQSAIDQITGKLNRLIEKTNQQFELIDNEFTEVEKQIGNLINWTKDSITEVWSYNAELIVAMENQHTIDLADSEMNRLYERVRKQLRENAEEDGTGCFEIFHKCDDDCMASIRNNTYDHSKYREEAMQNRIQIDPVKLSSGYKDVILWFSFGASCFLLLAIAMGLVFICVKNGNMRCTICI

SEQ ID NO: 73 - protein, 222 aa, Influenza virus A
  source 1..222: note = influenza A HA subtype H8 HA2 domain
GLFGAIAGFIEGGWSGMIDGWYGFHHSNSEGTGMAADQKSTQEAIDKITNKVNNIVDKMNREFEVVNHEFSEVEKRINMINDKIDDQIEDLWAYNAELLVLLENQKTLDEHDSNVKNLFDEVKRRLSANAIDAGNGCFDILHKCDNECMETIKNGTYDHKEYEEEAKLERSKINGVKLEENTTYKILSIYSTVAASLCLAILIAGGLILGMQNGSCRCMFCI

SEQ ID NO: 74 - protein, 222 aa, Influenza virus A
  source 1..222: note = influenza A HA subtype H9 HA2 domain
GLFGAIAGFIEGGWPGLVAGWYGFQHSNDQGVGMAADKGSTQKAIDKITSKVNNIIDKMNKQYEVIDHEFNELEARLNMINNKIDDQIQDIWAYNAELLVLLENQKTLDEHDANVNNLYNKVKRALGSNAVEDGNGCFELYHKCDDQCMETIRNGTYDRQKYQEESRLERQKIEGVKLESEGTYKILTIYSTVASSLVLAMGFAAFLFWAMSNGSCRCNICI

SEQ ID NO: 75 - protein, 221 aa, Influenza virus A
  source 1..221: note = influenza A HA subtype H10 HA2 domain
GLFGAIAGFIENGWEGMVDGWYGFRHQNAQGTGQAADYKSTQAAIDQITGKLNRLIEKTNTEFESIESEFSETEHQIGNVINWTKDSITDIWTYNAELLVAMENQHTIDMADSEMLNLYERVRKQLRQNAEEDGKGCFEIYHTCDDSCMESIRNNTYDHSQYREEALLNRLNINPVKLSSGYKDIILWFSFGESCFVLLAVVMGLVFFCLKNGNMRCTICI

SEQ ID NO: 76 - protein, 223 aa, Influenza virus A
  source 1..223: note = influenza A HA subtype H11 HA2 domain
GLFGAIAGFIEGGWPGLINGWYGFQHRDEEGTGIAADKESTQKAIDQITSKVNNIVDRMNTNFESVQHEFSEIEERINQLSKHVDDSVVDIWSYNAQLLVLLENEKTLDLHDSNVRNLHEKVRRMLKDNAKDEGNGCFTFYHKCDNKCIERVRNGTYDHKEFEEESKINRQEIEGVKLDSSGNVYKILSIYSCIASSLVLAALIMGFMFWACSNGSCRCTICI

SEQ ID NO: 77 - protein, 222 aa, Influenza virus A
  source 1..222: note = influenza A HA subtype H12 HA2 domain
GLFGAIAGFIEGGWPGLVAGWYGFQHQNAEGTGIAADRDSTQRAIDNMQNKLNNVIDKMNKQFEVVNHEFSEVESRINMINSKIDDQITDIWAYNAELLVLLENQKTLDEHDANVRNLHDRVRRVLRENAIDTGDGCFEILHKCDNNCMDTIRNGTYNHKEYEEESKIERQKVNGVKLEENSTYKILSIYSSVASSLVLLLMIIGGFIFGCQNGNVRCTFCI

SEQ ID NO: 78 - protein, 223 aa, Influenza virus A
  source 1..223: note = influenza A HA subtype H13 HA2 domain
GLFGAIAGFIEGGWPGLINGWYGFQHQNEQGTGIAADKESTQKAIDQITTKINNIIDKMNGNYDSIRGEFNQVEKRINMLADRIDDAVTDIWSYNAKLLVLLENDKTLDMHDANVKNLHEQVRRELKDNAIDEGNGCFELLHKCNDSCMETIRNGTYDHTEYAEESKLKRQEIDGIKLKSEDNVYKALSIYSCIASSVVLVGLILSFIMWACSSGNCRFNVCI

SEQ ID NO: 79 - protein, 221 aa, Influenza virus A
  source 1..221: note = influenza A HA subtype H14 HA2 domain
GLFGAIAGFIENGWQGLIDGWYGFRHQNAEGTGTAADLKSTQAAIDQINGKLNRLIEKTNEKYHQIEKEFEQVEGRIQDLEKYVEDTKIDLWSYNAELLVALENQHTIDVTDSEMNKLFERVRRQLRENAEDQGNGCFEIFHQCDNNCIESIRNGTYDHNIYRDEAINNRIKINPVTLTMGYKDIILWISFSMSCFVFVALILGFVLWACQNGNIRCQICI

SEQ ID NO: 80 - protein, 221 aa, Influenza virus A
  source 1..221: note = influenza A HA subtype H15 HA2 domain
GLFGAIAGFIENGWEGLIDGWYGFRHQNAQGQGTAADYKSTQAAIDQITGKLNRLIEKTNKQFELIDNEFTEVEQQIGNVINWTRDSLTEIWSYNAELLVAMENQHTIDLADSEMNKLYERVRRQLRENAEEDGTGCFEIFHRCDDQCMESIRNNTYNHTEYRQEALQNRIMINPVKLSSGYKDVILWFSFGASCVMLLAIAMGLIFMCVKNGNLRCTICI

SEQ ID NO: 81 - protein, 223 aa, Influenza virus A
  source 1..223: note = influenza A HA subtype H16 HA2 domain
GLFGAIAGFIEGGWPGLINGWYGFQHQNEQGTGIAADKASTQKAINEITTKINNIIEKMNGNYDSIRGEFNQVEKRINMLADRVDDAVTDIWSYNAKLLVLLENDRTLDLHDANVRNLHDQVKRALKSNAIDEGDGCFNLLHKCNDSCMETIRNGTYNHEDYREESQLKRQEIEGIKLKTEDNVYKVLSIYSCIASSIVLVGLILAFIMWACSNGSCRFNVCI

SEQ ID NO: 82 - protein, 180 aa, Influenza virus A
  source 1..180: note = influenza A HA2 domain subtype H1 stem domain
GLFGAIAGFIEGGWTGMIDGWYGYHHQNEQGSGYAADQKSTQNAINGITNKVNTVIEKMNIQFTAVGKEFNKLEKRMENLNKKVDDGFLDIWTYNAELLVLLENERTLDFHDSNVKNLYEKVKSQLKNNAKEIGNGCFEFYHKCDNECMESVRNGTYDYPKYSEESKLNREKVDGVKLES

SEQ ID NO: 83 - protein, 180 aa, Influenza virus A
  source 1..180: note = influenza A HA2 domain subtype H2 stem domain
GLFGAIAGFIEGGWQGMIDGWYGYHHSNDQGSGYAADKESTQKAIDGITNRVNSVIEKMNTQFEAVGKEFSNLEKRLENLNKKMEDGFLDVWTYNAELLVLMENERTLDFHDSNVKNLYDRVRMQLRDNAKELGNGCFEFYHKCDDECMNSVKNGTYDYPKYEEESKLNRNEIKGVKLSN

SEQ ID NO: 84 - protein, 179 aa, Influenza virus A
  source 1..179: note = influenza A HA2 domain subtype H3 stem domain
GLFGAIAGFIENGWEGMIDGWYGFRHQNSEGTGQAADLKSTQAAIDQINGKLNRVIEKTNEKFHQIEKEFSEVEGRIQDLEKYVEDTKIDLWSYNAELLVALENQHTIDLTDSEMNKLFEKTRRQLRENAEDMGNGCFKIYHKCDNACIESIRNGTYDHDVYRDEALNNRFQIKGVELK

SEQ ID NO: 85 - protein, 179 aa, Influenza virus A
  source 1..179: note = influenza A HA2 domain subtype H4 stem domain
GLFGAIAGFIENGWQGLIDGWYGFRHQNAEGTGTAADLKSTQAAIDQINGKLNRLIEKTNDKYHQIEKEFEQVEGRIQDLENYVEDTKIDLWSYNAELLVALENQHTIDVTDSEMNKLFERVRRQLRENAEDKGNGCFEIFHKCDNNCIESIRNGTYDHDIYRDEAINNRFQIQGVKLT

SEQ ID NO: 86 - protein, 180 aa, Influenza virus A
  source 1..180: note = influenza A HA2 domain subtype H5 stem domain
GLFGAIAGFIEGGWQGMVDGWYGYHHSNEQGSGYAADKESTQKAIDGITNKVNSIIDKMNTRFEAVGKEFNNLERRVENLNKKMEDGFLDVWTYNVELLVLMENERTLDFHDSNVNNLYDKVRLQLKDNARELGNGCFEFYHKCDNECMESVRNGTYDYPQYSEEARLNREEISGVKLES

SEQ ID NO: 87 - protein, 180 aa, Influenza virus A
  source 1..180: note = influenza A HA2 domain subtype H6 stem domain
GLFGAIAGFIEGGWTGMIDGWYGYHHENSQGSGYAADRESTQKAVDGITNKVNSIIDKMNTQFEAVDHEFSNLERRIDNLNKRMEDGFLDVWTYNAELLVLLENERTLDLHDANVKNLYERVKSQLRDNAMILGNGCFEFWHKCDDECMESVKNGTYDYPKYQDESKLNRQEIESVKLES

SEQ ID NO: 88 - protein, 179 aa, Influenza virus A
  source 1..179: note = influenza A HA2 domain subtype H7 stem domain
GLFGAIAGFIENGWEGLVDGWYGFRHQNAQGEGTAADYKSTQSAIDQITGKLNRLIEKTNQQFELIDNEFTEVEKQIGNLINWTKDSITEVWSYNAELIVAMENQHTIDLADSEMNRLYERVRKQLRENAEEDGTGCFEIFHKCDDDCMASIRNNTYDHSKYREEAMQNRIQIDPVKLS

SEQ ID NO: 89 - protein, 180 aa, Influenza virus A
  source 1..180: note = influenza A HA2 domain subtype H8 stem domain
GLFGAIAGFIEGGWSGMIDGWYGFHHSNSEGTGMAADQKSTQEAIDKITNKVNNIVDKMNREFEVVNHEFSEVEKRINMINDKIDDQIEDLWAYNAELLVLLENQKTLDEHDSNVKNLFDEVKRRLSANAIDAGNGCFDILHKCDNECMETIKNGTYDHKEYEEEAKLERSKINGVKLEE

SEQ ID NO: 90 - protein, 180 aa, Influenza virus A
  source 1..180: note = influenza A HA2 domain subtype H9 stem domain
GLFGAIAGFIEGGWPGLVAGWYGFQHSNDQGVGMAADKGSTQKAIDKITSKVNNIIDKMNKQYEVIDHEFNELEARLNMINNKIDDQIQDIWAYNAELLVLLENQKTLDEHDANVNNLYNKVKRALGSNAVEDGNGCFELYHKCDDQCMETIRNGTYDRQKYQEESRLERQKIEGVKLES

SEQ ID NO: 91 - protein, 179 aa, Influenza virus A
  source 1..179: note = influenza A HA2 domain subtype H10 stem domain
GLFGAIAGFIENGWEGMVDGWYGFRHQNAQGTGQAADYKSTQAAIDQITGKLNRLIEKTNTEFESIESEFSETEHQIGNVINWTKDSITDIWTYNAELLVAMENQHTIDMADSEMLNLYERVRKQLRQNAEEDGKGCFEIYHTCDDSCMESIRNNTYDHSQYREEALLNRLNINPVKLS

SEQ ID NO: 92 - protein, 181 aa, Influenza virus A
  source 1..181: note = influenza A HA2 domain subtype H11 stem domain
GLFGAIAGFIEGGWPGLINGWYGFQHRDEEGTGIAADKESTQKAIDQITSKVNNIVDRMNTNFESVQHEFSEIEERINQLSKHVDDSVVDIWSYNAQLLVLLENEKTLDLHDSNVRNLHEKVRRMLKDNAKDEGNGCFTFYHKCDNKCIERVRNGTYDHKEFEEESKINRQEIEGVKLDSS

SEQ ID NO: 93 - protein, 180 aa, Influenza virus A
  source 1..180: note = influenza A HA2 domain subtype H12 stem domain
GLFGAIAGFIEGGWPGLVAGWYGFQHQNAEGTGIAADRDSTQRAIDNMQNKLNNVIDKMNKQFEVVNHEFSEVESRINMINSKIDDQITDIWAYNAELLVLLENQKTLDEHDANVRNLHDRVRRVLRENAIDTGDGCFEILHKCDNNCMDTIRNGTYNHKEYEEESKIERQKVNGVKLEE

SEQ ID NO: 94 - protein, 181 aa, Influenza virus A
  source 1..181: note = influenza A HA2 domain subtype H13 stem domain
GLFGAIAGFIEGGWPGLINGWYGFQHQNEQGTGIAADKESTQKAIDQITTKINNIIDKMNGNYDSIRGEFNQVEKRINMLADRIDDAVTDIWSYNAKLLVLLENDKTLDMHDANVKNLHEQVRRELKDNAIDEGNGCFELLHKCNDSCMETIRNGTYDHTEYAEESKLKRQEIDGIKLKSE

SEQ ID NO: 95 - protein, 179 aa, Influenza virus A
  source 1..179: note = influenza A HA2 domain subtype H14 stem domain
GLFGAIAGFIENGWQGLIDGWYGFRHQNAEGTGTAADLKSTQAAIDQINGKLNRLIEKTNEKYHQIEKEFEQVEGRIQDLEKYVEDTKIDLWSYNAELLVALENQHTIDVTDSEMNKLFERVRRQLRENAEDQGNGCFEIFHQCDNNCIESIRNGTYDHNIYRDEAINNRIKINPVTLT

SEQ ID NO: 96 - protein, 179 aa, Influenza virus A
  source 1..179: note = influenza A HA2 domain subtype H15 stem domain
GLFGAIAGFIENGWEGLIDGWYGFRHQNAQGQGTAADYKSTQAAIDQITGKLNRLIEKTNKQFELIDNEFTEVEQQIGNVINWTRDSLTEIWSYNAELLVAMENQHTIDLADSEMNKLYERVRRQLRENAEEDGTGCFEIFHRCDDQCMESIRNNTYNHTEYRQEALQNRIMINPVKLS

SEQ ID NO: 97 - protein, 181 aa, Influenza virus A
  source 1..181: note = influenza A HA2 domain subtype H16 stem domain
GLFGAIAGFIEGGWPGLINGWYGFQHQNEQGTGIAADKASTQKAINEITTKINNIIEKMNGNYDSIRGEFNQVEKRINMLADRVDDAVTDIWSYNAKLLVLLENDRTLDLHDANVRNLHDQVKRALKSNAIDEGDGCFNLLHKCNDSCMETIRNGTYNHEDYREESQLKRQEIEGIKLKTE

SEQ ID NO: 98 - protein, 5 aa, Influenza virus A
  source 1..5: note = influenza A HA2 domain subtype H1 Luminal domain
MGIYQ

SEQ ID NO: 99 - protein, 5 aa, Influenza virus A
  source 1..5: note = influenza A HA2 domain subtype H2 Luminal domain
MGVYQ

SEQ ID NO: 100 - protein, 5 aa, Influenza virus A
  source 1..5: note = influenza A HA2 domain subtype H3 Luminal domain
SGYKD

SEQ ID NO: 101 - protein, 5 aa, Influenza virus A
  source 1..5: note = influenza A HA2 domain subtype H4 Luminal domain
QGYKD

SEQ ID NO: 102 - protein, 5 aa, Influenza virus A
  source 1..5: note = influenza A HA2 domain subtype H5 Luminal domain
MGVYQ

SEQ ID NO: 103 - protein, 5 aa, Influenza virus A
  source 1..5: note = influenza A HA2 domain subtype H6 Luminal domain
LGVYQ

SEQ ID NO: 104 - protein, 5 aa, Influenza virus A
  source 1..5: note = influenza A HA2 domain subtype H7 Luminal domain
SGYKD

SEQ ID NO: 105 - protein, 5 aa, Influenza virus A
  source 1..5: note = influenza A HA2 domain subtype H8 Luminal domain
NTTYK

SEQ ID NO: 106 - protein, 5 aa, Influenza virus A
  source 1..5: note = influenza A HA2 domain subtype H9 Luminal domain
EGTYK

SEQ ID NO: 107 - protein, 5 aa, Influenza virus A
  source 1..5: note = influenza A HA2 domain subtype H10 Luminal domain
SGYKD

SEQ ID NO: 108 - protein, 5 aa, Influenza virus A
  source 1..5: note = influenza A HA2 domain subtype H11 Luminal domain
GNVYK

SEQ ID NO: 109 - protein, 5 aa, Influenza virus A
  source 1..5: note = influenza A HA2 domain subtype H12 Luminal domain
NSTYK

SEQ ID NO: 110 - protein, 5 aa, Influenza virus A
  source 1..5: note = influenza A HA2 domain subtype H13 Luminal domain
DNVYK

SEQ ID NO: 111 - protein, 5 aa, Influenza virus A
  source 1..5: note = influenza A HA2 domain subtype H14 Luminal domain
MGYKD

SEQ ID NO: 112 - protein, 5 aa, Influenza virus A
  source 1..5: note = influenza A HA2 domain subtype H15 Luminal domain
SGYKD

SEQ ID NO: 113 - protein, 5 aa, Influenza virus A
  source 1..5: note = influenza A HA2 domain subtype H16 Luminal domain
DNVYK

SEQ ID NO: 114 - protein, 27 aa, Influenza virus A
  source 1..27: note = influenza A HA2 domain subtype H1 transmembrane domain
ILAIYSTVASSLVLLVSLGAISFWMCS

SEQ ID NO: 115 - protein, 27 aa, Influenza virus A
  source 1..27: note = influenza A HA2 domain subtype H2 transmembrane domain
ILAIYATVAGSLSLAIMIAGISLWMCS

SEQ ID NO: 116 - protein, 27 aa, Influenza virus A
  source 1..27: note = influenza A HA2 domain subtype H3 transmembrane domain
WILWISFAISCFLLCVVLLGFIMWACQ

SEQ ID NO: 117 - protein, 27 aa, Influenza virus A
  source 1..27: note = influenza A HA2 domain subtype H4 transmembrane domain
IILWISFSISCFLLVALLLAFILWACQ

SEQ ID NO: 118 - protein, 27 aa, Influenza virus A
  source 1..27: note = influenza A HA2 domain subtype H5 transmembrane domain
ILSIYSTVASSLALAIMIAGLSFWMCS

SEQ ID NO: 119 - protein, 27 aa, Influenza virus A
  source 1..27: note = influenza A HA2 domain subtype H6 transmembrane domain
ILAIYSTVSSSLVLVGLIIAVGLWMCS

SEQ ID NO: 120 - protein, 27 aa, Influenza virus A
  source 1..27: note = influenza A HA2 domain subtype H7 transmembrane domain
VILWFSFGASCFLLLAIAMGLVFICVK

SEQ ID NO: 121 - protein, 27 aa, Influenza virus A
  source 1..27: note = influenza A HA2 domain subtype H8 transmembrane domain
ILSIYSTVAASLCLAILIAGGLILGMQ

SEQ ID NO: 122 - protein, 27 aa, Influenza virus A
  source 1..27: note = influenza A HA2 domain subtype H9 transmembrane domain
ILTIYSTVASSLVLAMGFAAFLFWAMS

SEQ ID NO: 123 - protein, 27 aa, Influenza virus A
  source 1..27: note = influenza A HA2 domain subtype H10 transmembrane domain
IILWFSFGESCFVLLAVVMGLVFFCLK

SEQ ID NO: 124 - protein, 27 aa, Influenza virus A
  source 1..27: note = influenza A HA2 domain subtype H11 transmembrane domain
ILSIYSCIASSLVLAALIMGFMFWACS

SEQ ID NO: 125 - protein, 28 aa, Influenza virus A
  source 1..28: note = influenza A HA2 domain subtype H12 transmembrane domain
ILSIYSSVASSLVLLLMIIGGFIFGCQN

SEQ ID NO: 126 - protein, 28 aa, Influenza virus A
  source 1..28: note = influenza A HA2 domain subtype H13 transmembrane domain
ALSIYSCIASSVVLVGLILSFIMWACSS

SEQ ID NO: 127 - protein, 27 aa, Influenza virus A
  source 1..27: note = influenza A HA2 domain subtype H14 transmembrane domain
IILWISFSMSCFVFVALILGFVLWACQ

SEQ ID NO: 128 - protein, 28 aa, Influenza virus A
  source 1..28: note = influenza A HA2 domain subtype H15 transmembrane domain
VILWFSFGASCVMLLAIAMGLIFMCVKN

SEQ ID NO: 129 - protein, 27 aa, Influenza virus A
  source 1..27: note = influenza A HA2 domain subtype H16 transmembrane domain
VLSIYSCIASSIVLVGLILAFIMWACS

SEQ ID NO: 130 - protein, 10 aa, Influenza virus A
  source 1..10: note = influenza A HA2 domain subtype H1 cytoplasmic domain
NGSLQCRICI

SEQ ID NO: 131 - protein, 10 aa, Influenza virus A
  source 1..10: note = influenza A HA2 domain subtype H2 cytoplasmic domain
NGSLQCRICI

SEQ ID NO: 132 - protein, 10 aa, Influenza virus A
  source 1..10: note = influenza A HA2 domain subtype H3 cytoplasmic domain
RGNIRCNICI

SEQ ID NO: 133 - protein, 10 aa, Influenza virus A
  source 1..10: note = influenza A HA2 domain subtype H4 cytoplasmic domain
NGNIRCQICI

SEQ ID NO: 134 - protein, 10 aa, Influenza virus A
  source 1..10: note = influenza A HA2 domain subtype H5 cytoplasmic domain
NGSLQCRICI

SEQ ID NO: 135 - protein, 10 aa, Influenza virus A
  source 1..10: note = influenza A HA2 domain subtype H6 cytoplasmic domain
NGSMQCRICI

SEQ ID NO: 136 - protein, 10 aa, Influenza virus A
  source 1..10: note = influenza A HA2 domain subtype H7 cytoplasmic domain
NGNMRCTICI

SEQ ID NO: 137 - protein, 10 aa, Influenza virus A
  source 1..10: note = influenza A HA2 domain subtype H8 cytoplasmic domain
NGSCRCMFCI

SEQ ID NO: 138 - protein, 10 aa, Influenza virus A
  source 1..10: note = influenza A HA2 domain subtype H9 cytoplasmic domain
NGSCRCNICI

SEQ ID NO: 139 - protein, 10 aa, Influenza virus A
  source 1..10: note = influenza A HA2 domain subtype H10 cytoplasmic domain
NGNMRCTICI

SEQ ID NO: 140 - protein, 10 aa, Influenza virus A
  source 1..10: note = influenza A HA2 domain subtype H11 cytoplasmic domain
NGSCRCTICI

SEQ ID NO: 141 - protein, 9 aa, Influenza virus A
  source 1..9: note = influenza A HA2 domain subtype H12 cytoplasmic domain
GNVRCTFCI

SEQ ID NO: 142 - protein, 9 aa, Influenza virus A
  source 1..9: note = influenza A HA2 domain subtype H13 cytoplasmic domain
GNCRFNVCI

SEQ ID NO: 143 - protein, 10 aa, Influenza virus A
  source 1..10: note = influenza A HA2 domain subtype H14 cytoplasmic domain
NGNIRCQICI

SEQ ID NO: 144 - protein, 9 aa, Influenza virus A
  source 1..9: note = influenza A HA2 domain subtype H15 cytoplasmic domain
GNLRCTICI

SEQ ID NO: 145 - protein, 10 aa, Influenza virus A
  source 1..10: note = influenza A HA2 domain subtype H16 cytoplasmic domain
NGSCRFNVCI

SEQ ID NO: 146-148 - skipped (3 entries)

SEQ ID NO: 149 - protein, 19 aa, synthetic construct
  VARIANT 1: note = Xaa = Lys, Gln, Arg, Leu or Tyr
  VARIANT 11: note = Xaa = Ile, Val or Met
  VARIANT 12: note = Xaa = Thr, Gln or Asn
  VARIANT 15: note = Xaa = Val or Leu
  VARIANT 18: note = Xaa = Val, Ile or Leu
  VARIANT 19: note = Xaa = Val or Ile
  source 1..19: note = sequence of HA2 domain
  VARIANT 2..3: note = Xaa = any amino acid
  VARIANT 6: note = Xaa = any amino acid
  VARIANT 10: note = Xaa = any amino acid
  VARIANT 13: note = Xaa = any amino acid
  VARIANT 17: note = Xaa = any amino acid
XXXTQXAIDXXXXKXNXXX

SEQ ID NO: 150 - protein, 15 aa, Influenza virus B
  source 1..15: note = Signal peptide of Influenza B HA construct variant Arg50-Ser277
MKAIIVILMVVTSNA

SEQ ID NO: 151 - protein, 15 aa, Influenza virus B
  source 1..15: note = Signal peptide of Influenza B HA construct variant Ala66-Trp271
MKAIIVILMVVTSNA

SEQ ID NO: 152 - protein, 15 aa, Influenza virus B
  source 1..15: note = Signal peptide of Influenza B HA construct variant Lys80-Ser277
MKAIIVILMVVTSNA

SEQ ID NO: 153 - protein, 15 aa, Influenza virus B
  source 1..15: note = Signal peptide of Influenza B HA construct variant Arg80-Ser277
MKAIIVILMVVTSNA

SEQ ID NO: 154 - protein, 50 aa, Influenza virus B
  source 1..50: note = HA1 N-terminal Stem Segment of Influenza B HA construct variant Arg50-Ser277
DRICTGITSSNSPHVVKTATQGEVNVTGVIPLTTTPTKSHFANLKGTETR

SEQ ID NO: 155 - protein, 66 aa, Influenza virus B
  source 1..66: note = HA1 N-terminal Stem Segment of Influenza B HA construct variant Ala66-Trp271
DRICTGITSSNSPHVVKTATQGEVNVTGVIPLTTTPTKSHFANLKGTETRGKLCPKCLNCTDLDVA

SEQ ID NO: 156 - protein, 80 aa, Influenza virus B
  source 1..80: note = HA1 N-terminal Stem Segment of Influenza B HA construct variant Lys80-Ser277
DRICTGITSSNSPHVVKTATQGEVNVTGVIPLTTTPTKSHFANLKGTETRGKLCPKCLNCTDLDVALGRPKCTGKIPSAK

SEQ ID NO: 157 - protein, 80 aa, Influenza virus B
  source 1..80: note = HA1 N-terminal Stem Segment of Influenza B HA construct variant Arg80-Ser277
DRICTGITSSNSPHVVKTATQGEVNVTGVIPLTTTPTKSHFANLKGTETRGKLCPKCLNCTDLDVALGRPKCTGKIPSAR

SEQ ID NO: 158 - protein, 68 aa, Influenza virus B
  source 1..68: note = HA1 C-terminal Stem Segment of Influenza B HA construct variant Arg50-Ser277
SKVIKGSLPLIGEADCLHEKYGGLNKSKPYYTGEHAKAIGNCPIWVKTPLKLANGTKYRPPAKLLKER

SEQ ID NO: 159 - protein, 74 aa, Influenza virus B
  source 1..74: note = HA1 C-terminal Stem Segment of Influenza B HA construct variant Ala66-Trp271
WCASGRSKVIKGSLPLIGEADCLHEKYGGLNKSKPYYTGEHAKAIGNCPIWVKTPLKLANGTKYRPPAKLLKER

SEQ ID NO: 160 - protein, 223 aa, Influenza virus B
  source 1..223: note = HA2 Domain of Influenza B HA construct variant Arg50-Ser277 and other variants listed in Table 3
GFFGAIAGFLEGGWEGMIAGWHGYTSHGAHGVAVAADLKSTQEAINKITKNLNSLSELEVKNLQRLSGAMDELHNEILELDEKVDDLRADTISSQIELAVLLSNEGIINSEDEHLLALERKLKKMLGPSAVEIGNGCFETKHKCNQTCLDRIAAGTFDAGEFSLPTFDSLNITAASLNDDGLDNHTILLYYSTAASSLAVTLMIAIFVVYMVSRDNVSCSICL

SEQ ID NO: 161 - protein, 179 aa, Influenza virus B
  source 1..179: note = Stem domain of Influenza B HA2 domain subtype HA2
GFFGAIAGFLEGGWEGMIAGWHGYTSHGAHGVAVAADLKSTQEAINKITKNLNSLSELEVKNLQRLSGAMDELHNEILELDEKVDDLRADTISSQIELAVLLSNEGIINSEDEHLLALERKLKKMLGPSAVEIGNGCFETKHKCNQTCLDRIAAGTFDAGEFSLPTFDSLNITAASLND

SEQ ID NO: 162 - protein, 5 aa, Influenza virus B
  source 1..5: note = luminal domain of Influenza B HA2 domain subtype HA2
DGLDN

SEQ ID NO: 163 - protein, 28 aa, Influenza virus B
  source 1..28: note = transmembrane domain of Influenza B HA2 domain subtype HA2
HTILLYYSTAASSLAVTLMIAIFVVYMV

SEQ ID NO: 164 - protein, 11 aa, Influenza virus B
  source 1..11: note = cytoplasmic domain of Influenza B HA2 domain subtype HA2
SRDNVSCSICL

SEQ ID NO: 165 - protein, 23 aa, synthetic construct
  source 1..23: note = turn loop linker sequence
ITPNGSIPNDKPFQNVNKITYGA

SEQ ID NO: 166 - protein, 6 aa, synthetic construct
  source 1..6: note = His tag
HHHHHH

SEQ ID NO: 167 - protein, 29 aa, synthetic construct
  source 1..29: note = example of a foldon domain
GSGYIPEAPRDGQAYVRKDGEWVLLSTFL

SEQ ID NO: 168 - protein, 7 aa, synthetic construct
  source 1..7: note = thrombin cleavage site
LVPRGSP

SEQ ID NO: 169-176 - skipped (8 entries)

SEQ ID NO: 177 - protein, 41 aa, Influenza virus A
  source 1..41: note = N-terminal stem segment of Influenza A HA subtype H1(no Cys) Short Stem Domain sequence
DTICIGYHANNSTDTVDTVLEKNVTVTHSVNLLEDSHNGKL

SEQ ID NO: 178 - protein, 41 aa, Influenza virus A; identical to SEQ ID NO: 177
  source 1..41: note = N-terminal stem segment of Influenza A HA subtype H1(no Cys-delta 1) Short Stem Domain sequence

SEQ ID NO: 179 - protein, 40 aa, Influenza virus A
  source 1..40: note = N-terminal stem segment of Influenza A HA subtype H1(no Cys-delta 3) Short Stem Domain sequence
DTICIGYHANNSTDTVDTVLEKNVTVTHSVNLLEDSHNGK

SEQ ID NO: 180 - protein, 41 aa, Influenza virus A
  source 1..41: note = N-terminal stem segment of Influenza A HA subtype H2(no Cys) Short Stem Domain sequence
DQICIGYHSNNSTEKVDTILERNVTVTHAQNILEKTHNGKL

SEQ ID NO: 181 - protein, 41 aa, Influenza virus A; identical to SEQ ID NO: 180
  source 1..41: note = N-terminal stem segment of Influenza A HA subtype H2(no Cys-delta 1) Short Stem Domain sequence

SEQ ID NO: 182 - protein, 40 aa, Influenza virus A
  source 1..40: note = N-terminal stem segment of Influenza A HA subtype H2(no Cys-delta 3) Short Stem Domain sequence
DQICIGYHSNNSTEKVDTILERNVTVTHAQNILEKTHNGK

SEQ ID NO: 183 - protein, 51 aa, Influenza virus A
  source 1..51: note = N-terminal stem segment of Influenza A HA subtype H3(no Cys) Short Stem Domain sequence
QDLPGNDNSTATLCLGHHAVPNGTLVKTITDDQIEVTNATELVQSSSTGKI

SEQ ID NO: 184 - protein, 51 aa, Influenza virus A; identical to SEQ ID NO: 183
  source 1..51: note = N-terminal stem segment of Influenza A HA subtype H3(no Cys-delta 1) Short Stem Domain sequence

SEQ ID NO: 185 - protein, 50 aa, Influenza virus A
  source 1..50: note = N-terminal stem segment of Influenza A HA subtype H3(no Cys-delta 3) Short Stem Domain sequence
QDLPGNDNSTATLCLGHHAVPNGTLVKTITDDQIEVTNATELVQSSSTGK

SEQ ID NO: 186 - protein, 47 aa, Influenza virus A
  source 1..47: note = N-terminal stem segment of Influenza A HA subtype H4(no Cys) Short Stem Domain sequence
QNYTGNPVICMGHHAVANGTMVKTLADDQVEVVTAQELVESQNLPEL

SEQ ID NO: 187 - protein, 47 aa, Influenza virus A; identical to SEQ ID NO: 186
  source 1..47: note = N-terminal stem segment of Influenza A HA subtype H4(no Cys-delta 1) Short Stem Domain sequence

SEQ ID NO: 188 - protein, 46 aa, Influenza virus A
  source 1..46: note = N-terminal stem segment of Influenza A HA subtype H4(no Cys-delta 3) Short Stem Domain sequence
QNYTGNPVICMGHHAVANGTMVKTLADDQVEVVTAQELVESQNLPE

SEQ ID NO: 189 - protein, 41 aa, Influenza virus A
  source 1..41: note = N-terminal stem segment of Influenza A HA subtype H5(no Cys) Short Stem Domain sequence
DQICIGYHANKSTKQVDTIMEKNVTVTHAQDILERTHNGKL

SEQ ID NO: 190 - protein, 41 aa, Influenza virus A; identical to SEQ ID NO: 189
  source 1..41: note = N-terminal stem segment of Influenza A HA subtype H5(no Cys-delta 1) Short Stem Domain sequence

SEQ ID NO: 191 - protein, 40 aa, Influenza virus A
  source 1..40: note = N-terminal stem segment of Influenza A HA subtype H5(no Cys-delta 3) Short Stem Domain sequence
DQICIGYHANKSTKQVDTIMEKNVTVTHAQDILERTHNGK

SEQ ID NO: 192 - protein, 41 aa, Influenza virus A
  source 1..41: note = N-terminal stem segment of Influenza A HA subtype H6(no Cys) Short Stem Domain sequence
DKICIGYHANNSTTQIDTILEKNVTVTHSVELLENQKEERF

SEQ ID NO: 193 - protein, 41 aa, Influenza virus A; identical to SEQ ID NO: 192
  source 1..41: note = N-terminal stem segment of Influenza A HA subtype H6(no Cys-delta 1) Short Stem Domain sequence

SEQ ID NO: 194 - protein, 40 aa, Influenza virus A
  source 1..40: note = N-terminal stem segment of Influenza A HA subtype H6(no Cys-delta 3) Short Stem Domain sequence
DKICIGYHANNSTTQIDTILEKNVTVTHSVELLENQKEER

SEQ ID NO: 195 - protein, 41 aa, Influenza virus A
  source 1..41: note = N-terminal stem segment of Influenza A HA subtype H7(no Cys) Short Stem Domain sequence
DKICLGHHAVSNGTKVNTLTERGVEVVNATETVERTNIPKI

SEQ ID NO: 196 - protein, 41 aa, Influenza virus A; identical to SEQ ID NO: 195
  source 1..41: note = N-terminal stem segment of Influenza A HA subtype H7(no Cys-delta 1) Short Stem Domain sequence

SEQ ID NO: 197 - protein, 40 aa, Influenza virus A
  source 1..40: note = N-terminal stem segment of Influenza A HA subtype H7(no Cys-delta 3) Short Stem Domain sequence
DKICLGHHAVSNGTKVNTLTERGVEVVNATETVERTNIPK

SEQ ID NO: 198 - protein, 41 aa, Influenza virus A
  source 1..41: note = N-terminal stem segment of Influenza A HA subtype H8(no Cys) Short Stem Domain sequence
DRICIGYQSNNSTDTVNTLIEQNVPVTQTMELVETEKHPAY

SEQ ID NO: 199 - protein, 41 aa, Influenza virus A; identical to SEQ ID NO: 198
  source 1..41: note = N-terminal stem segment of Influenza A HA subtype H8(no Cys-delta 1) Short Stem Domain sequence

SEQ ID NO: 200 - protein, 40 aa, Influenza virus A
  source 1..40: note = N-terminal stem segment of Influenza A HA subtype H8(no Cys-delta 3) Short Stem Domain sequence
DRICIGYQSNNSTDTVNTLIEQNVPVTQTMELVETEKHPA

SEQ ID NO: 201 - protein, 41 aa, Influenza virus A
  source 1..41: note = N-terminal stem segment of Influenza A HA subtype H9(no Cys) Short Stem Domain sequence
DKICIGYQSTNSTETVDTLTESNVPVTHTKELLHTEHNGML

SEQ ID NO: 202 - protein, 41 aa, Influenza virus A; identical to SEQ ID NO: 201
  source 1..41: note = N-terminal stem segment of Influenza A HA subtype H9(no Cys-delta 1) Short Stem Domain sequence

SEQ ID NO: 203 - protein, 40 aa, Influenza virus A
  source 1..40: note = N-terminal stem segment of Influenza A HA subtype H9(no Cys-delta 3) Short Stem Domain sequence
DKICIGYQSTNSTETVDTLTESNVPVTHTKELLHTEHNGM

SEQ ID NO: 204 - protein, 42 aa, Influenza virus A
  source 1..42: note = N-terminal stem segment of Influenza A HA subtype H10(no Cys) Short Stem Domain sequence
LDRICLGHHAVANGTIVKTLTNEQEEVTNATETVESTNLNKL

SEQ ID NO: 205 - protein, 42 aa, Influenza virus A; identical to SEQ ID NO: 204
  source 1..42: note = N-terminal stem segment of Influenza A HA subtype H10(no Cys-delta 1) Short Stem Domain sequence

SEQ ID NO: 206 - protein, 41 aa, Influenza virus A
  source 1..41: note = N-terminal stem segment of Influenza A HA subtype H10(no Cys-delta 3) Short Stem Domain sequence
LDRICLGHHAVANGTIVKTLTNEQEEVTNATETVESTNLNK

SEQ ID NO: 207 - protein, 41 aa, Influenza virus A
  source 1..41: note = N-terminal stem segment of Influenza A HA subtype H11(no Cys) Short Stem Domain sequence
DEICIGYLSNNSTDKVDTIIENNVTVTSSVELVETEHTGSF

SEQ ID NO: 208 - protein, 41 aa, Influenza virus A; identical to SEQ ID NO: 207
  source 1..41: note = N-terminal stem segment of Influenza A HA subtype H11(no Cys-delta 1) Short Stem Domain sequence

SEQ ID NO: 209 - protein, 40 aa, Influenza virus A
  source 1..40: note = N-terminal stem segment of Influenza A HA subtype H11(no Cys-delta 3) Short Stem Domain sequence
DEICIGYLSNNSTDKVDTIIENNVTVTSSVELVETEHTGS

SEQ ID NO: 210 - protein, 41 aa, Influenza virus A
  source 1..41: note = N-terminal stem segment of Influenza A HA subtype H12(no Cys) Short Stem Domain sequence
DKICIGYQTNNSTETVNTLSEQNVPVTQVEELVHRGIDPIL

SEQ ID NO: 211 - protein, 41 aa, Influenza virus A; identical to SEQ ID NO: 210
  source 1..41: note = N-terminal stem segment of Influenza A HA subtype H12(no Cys-delta 1) Short Stem Domain sequence

SEQ ID NO: 212 - protein, 40 aa, Influenza virus A
  source 1..40: note = N-terminal stem segment of Influenza A HA subtype H12(no Cys-delta 3) Short Stem Domain sequence
DKICIGYQTNNSTETVNTLSEQNVPVTQVEELVHRGIDPI

SEQ ID NO: 213 - protein, 41 aa, Influenza virus A
  source 1..41: note = N-terminal stem segment of Influenza A HA subtype H13(no Cys) Short Stem Domain sequence
DRICVGYLSTNSSERVDTLLENGVPVTSSIDLIETNHTGTY

SEQ ID NO: 214 - protein, 41 aa, Influenza virus A; identical to SEQ ID NO: 213
  source 1..41: note = N-terminal stem segment of Influenza A HA subtype H13(no Cys-delta 1) Short Stem Domain sequence

SEQ ID NO: 215 - protein, 40 aa, Influenza virus A
  source 1..40: note = N-terminal stem segment of Influenza A HA subtype H13(no Cys-delta 3) Short Stem Domain sequence
DRICVGYLSTNSSERVDTLLENGVPVTSSIDLIETNHTGT

SEQ ID NO: 216 - protein, 50 aa, Influenza virus A
  source 1..50: note = N-terminal stem segment of Influenza A HA subtype H14(no Cys) Short Stem Domain sequence
QITNGTTGNPIICLGHHAVENGTSVKTLTDNHVEVVSAKELVETNHTDEL

SEQ ID NO: 217 - protein, 50 aa, Influenza virus A; identical to SEQ ID NO: 216
  source 1..50: note = N-terminal stem segment of Influenza A HA subtype H14(no Cys-delta 1) Short Stem Domain sequence

SEQ ID NO: 218 - protein, 49 aa, Influenza virus A
  source 1..49: note = N-terminal stem segment of Influenza A HA subtype H14(no Cys-delta 3) Short Stem Domain sequence
QITNGTTGNPIICLGHHAVENGTSVKTLTDNHVEVVSAKELVETNHTDE

SEQ ID NO: 219 - protein, 41 aa, Influenza virus A
  source 1..41: note = N-terminal stem segment of Influenza A HA subtype H15(no Cys) Short Stem Domain sequence
DKICLGHHAVANGTKVNTLTERGVEVVNATETVEITGIDKV

SEQ ID NO: 220 - protein, 41 aa, Influenza virus A; identical to SEQ ID NO: 219
  source 1..41: note = N-terminal stem segment of Influenza A HA subtype H15(no Cys-delta 1) Short Stem Domain sequence

SEQ ID NO: 221 - protein, 40 aa, Influenza virus A
  source 1..40: note = N-terminal stem segment of Influenza A HA subtype H15(no Cys-delta 3) Short Stem Domain sequence
DKICLGHHAVANGTKVNTLTERGVEVVNATETVEITGIDK

SEQ ID NO: 222 - protein, 41 aa, Influenza virus A
  source 1..41: note = N-terminal stem segment of Influenza A HA subtype H16(no Cys) Short Stem Domain sequence
DKICIGYLSNNSSDTVDTLTENGVPVTSSVDLVETNHTGTY

SEQ ID NO: 223 - protein, 41 aa, Influenza virus A; identical to SEQ ID NO: 222
  source 1..41: note = N-terminal stem segment of Influenza A HA subtype H16(no Cys-delta 1) Short Stem Domain sequence

SEQ ID NO: 224 - protein, 40 aa, Influenza virus A
  source 1..40: note = N-terminal stem segment of Influenza A HA subtype H16(no Cys-delta 3) Short Stem Domain sequence
DKICIGYLSNNSSDTVDTLTENGVPVTSSVDLVETNHTGT

SEQ ID NO: 225 - skipped

SEQ ID NO: 226 - protein, 52 aa, Influenza virus A
  source 1..52: note = C-terminal stem segment of Influenza A HA subtype H1(no Cys)
NTKCQTPLGAINSSLPYQNIHPVTIGECPKYVRSAKLRMVTGLRNNPSIQSR

SEQ ID NO: 227 - protein, 51 aa, Influenza virus A
  source 1..51: note = C-terminal stem segment of Influenza A HA subtype H1(no Cys-delta 1)
TKCQTPLGAINSSLPYQNIHPVTIGECPKYVRSAKLRMVTGLRNNPSIQSR

SEQ ID NO: 228 - protein, 50 aa, Influenza virus A
  source 1..50: note = C-terminal stem segment of Influenza A HA subtype H1(no Cys-delta 3)
KCQTPLGAINSSLPYQNIHPVTIGECPKYVRSAKLRMVTGLRNNPSIQSR

SEQ ID NO: 229 - protein, 52 aa, Influenza virus A
  source 1..52: note = C-terminal stem segment of Influenza A HA subtype H2(no Cys)
ETKCQTPLGAINTTLPFHNVHPLTIGECPKYVKSERLVLATGLRNVPQIESR

SEQ ID NO: 230 - protein, 51 aa, Influenza virus A
  source 1..51: note = C-terminal stem segment of Influenza A HA subtype H2(no Cys-delta 1)
TKCQTPLGAINTTLPFHNVHPLTIGECPKYVKSERLVLATGLRNVPQIESR

SEQ ID NO: 231 - protein, 50 aa, Influenza virus A
  source 1..50: note = C-terminal stem segment of Influenza A HA subtype H2(no Cys-delta 3)
KCQTPLGAINTTLPFHNVHPLTIGECPKYVKSERLVLATGLRNVPQIESR

SEQ ID NO: 232 - protein, 52 aa, Influenza virus A
  source 1..52: note = C-terminal stem segment of Influenza A HA subtype H3(no Cys)
ISECITPNGSIPNDKPFQNVNKITYGACPKYVKQNTLKLATGMRNVPEKQTR

SEQ ID NO: 233 - protein, 51 aa, Influenza virus A
  source 1..51: note = C-terminal stem segment of Influenza A HA subtype H3(no Cys-delta 1)
SECITPNGSIPNDKPFQNVNKITYGACPKYVKQNTLKLATGMRNVPEKQTR

SEQ ID NO: 234 - protein, 50 aa, Influenza virus A
  source 1..50: note = C-terminal stem segment of Influenza A HA subtype H3(no Cys-delta 3)
ECITPNGSIPNDKPFQNVNKITYGACPKYVKQNTLKLATGMRNVPEKQTR

SEQ ID NO: 235 - protein, 52 aa, Influenza virus A
  source 1..52: note = C-terminal stem segment of Influenza A HA subtype H4(no Cys)
VSKCHTDKGSLSTTKPFQNISRIAVGDCPRYVKQGSLKLATGMRNIPEKASR

SEQ ID NO: 236 - protein, 51 aa, Influenza virus A
  source 1..51: note = C-terminal stem segment of Influenza A HA subtype H4(no Cys-delta 1)
SKCHTDKGSLSTTKPFQNISRIAVGDCPRYVKQGSLKLATGMRNIPEKASR

SEQ ID NO: 237 - protein, 50 aa, Influenza virus A
  source 1..50: note = C-terminal stem segment of Influenza A HA subtype H4(no Cys-delta 3)
KCHTDKGSLSTTKPFQNISRIAVGDCPRYVKQGSLKLATGMRNIPEKASR

SEQ ID NO: 238 - protein, 52 aa, Influenza virus A
  source 1..52: note = C-terminal stem segment of Influenza A HA subtype H5(no Cys)
DTKCQTPVGEINSSMPFHNIHPHTIGECPKYVKSDRLVLATGLRNVPQRKKR

SEQ ID NO: 239 - protein, 51 aa, Influenza virus A
  source 1..51: note = C-terminal stem segment of Influenza A HA subtype H5(no Cys-delta 1)
TKCQTPVGEINSSMPFHNIHPHTIGECPKYVKSDRLVLATGLRNVPQRKKR

SEQ ID NO: 240 - protein, 50 aa, Influenza virus A
  source 1..50: note = C-terminal stem segment of Influenza A HA subtype H5(no Cys-delta 3)
KCQTPVGEINSSMPFHNIHPHTIGECPKYVKSDRLVLATGLRNVPQRKKR

SEQ ID NO: 241 - protein, 52 aa, Influenza virus A
  source 1..52: note = C-terminal stem segment of Influenza A HA subtype H6(no Cys)
DATCQTVAGVLRTNKTFQNVSPLWIGECPKYVKSESLRLATGLRNVPQIETR

SEQ ID NO: 242 - protein, 51 aa, Influenza virus A
  source 1..51: note = C-terminal stem segment of Influenza A HA subtype H6(no Cys-delta 1)
ATCQTVAGVLRTNKTFQNVSPLWIGECPKYVKSESLRLATGLRNVPQIETR

SEQ ID NO: 243 - protein, 50 aa, Influenza virus A
  source 1..50: note = C-terminal stem segment of Influenza A HA subtype H6(no Cys-delta 3)
TCQTVAGVLRTNKTFQNVSPLWIGECPKYVKSESLRLATGLRNVPQIETR

SEQ ID NO: 244 - protein, 56 aa, Influenza virus A
  source 1..56: note = C-terminal stem segment of Influenza A HA subtype H7(no Cys)
EGECYHSGGTITSRLPFQNINSRAVGKCPRYVKQESLLLATGMKNVPEPSKKRKKR

SEQ ID NO: 245 - protein, 55 aa, Influenza virus A
  source 1..55: note = C-terminal stem segment of Influenza A HA subtype H7(no Cys-delta 1)
GECYHSGGTITSRLPFQNINSRAVGKCPRYVKQESLLLATGMKNVPEPSKKRKKR

SEQ ID NO: 246 - protein, 54 aa, Influenza virus A
  source 1..54: note = C-terminal stem segment of Influenza A HA subtype H7(no Cys-delta 3)
ECYHSGGTITSRLPFQNINSRAVGKCPRYVKQESLLLATGMKNVPEPSKKRKKR

SEQ ID NO: 247 - protein, 52 aa, Influenza virus A
  source 1..52: note = C-terminal stem segment of Influenza A HA subtype H8(no Cys)
NTKCQTYAGAINSSKPFQNASRHYMGECPKYVKKASLRLAVGLRNTPSVEPR

SEQ ID NO: 248 - protein, 51 aa, Influenza virus A
  source 1..51: note = C-terminal stem segment of Influenza A HA subtype H8(no Cys-delta 1)
TKCQTYAGAINSSKPFQNASRHYMGECPKYVKKASLRLAVGLRNTPSVEPR

SEQ ID NO: 249 - protein, 50 aa, Influenza virus A
  source 1..50: note = C-terminal stem segment of Influenza A HA subtype H8(no Cys-delta 3)
KCQTYAGAINSSKPFQNASRHYMGECPKYVKKASLRLAVGLRNTPSVEPR

SEQ ID NO: 250 - protein, 52 aa, Influenza virus A
  source 1..52: note = C-terminal stem segment of Influenza A HA subtype H9(no Cys)
VVQCQTEKGGLNTTLPFHNISKYAFGNCPKYVGVKSLKLPVGLRNVPAVSSR

SEQ ID NO: 251 - protein, 51 aa, Influenza virus A
  source 1..51: note = C-terminal stem segment of Influenza A HA subtype H9(no Cys-delta 1)
VQCQTEKGGLNTTLPFHNISKYAFGNCPKYVGVKSLKLPVGLRNVPAVSSR

SEQ ID NO: 252 - protein, 50 aa, Influenza virus A
  source 1..50: note = C-terminal stem segment of Influenza A HA subtype H9(no Cys-delta 3)
QCQTEKGGLNTTLPFHNISKYAFGNCPKYVGVKSLKLPVGLRNVPAVSSR

SEQ ID NO: 253 - protein, 53 aa, Influenza virus A
  source 1..53: note = C-terminal stem segment of Influenza A HA subtype H10(no Cys)
ESKCFWRGGSINTKLPFQNLSPRTVGQCPKYVNQRSLLLATGMRNVPEVVQGR

SEQ ID NO: 254 - protein, 52 aa, Influenza virus A
  source 1..52: note = C-terminal stem segment of Influenza A HA subtype H10(no Cys-delta 1)
SKCFWRGGSINTKLPFQNLSPRTVGQCPKYVNQRSLLLATGMRNVPEVVQGR

SEQ ID NO: 255 - protein, 51 aa, Influenza virus A
  source 1..51: note = C-terminal stem segment of Influenza A HA subtype H10(no Cys-delta 3)
KCFWRGGSINTKLPFQNLSPRTVGQCPKYVNQRSLLLATGMRNVPEVVQGR

SEQ ID NO: 256 - protein, 52 aa, Influenza virus A
  source 1..52: note = C-terminal stem segment of Influenza A HA subtype H11(no Cys)
STKCQTEIGGINTNKSFHNVHRNTIGDCPKYVNVKSLKLATGPRNVPAIASR

SEQ ID NO: 257 - protein, 51 aa, Influenza virus A
  source 1..51: note = C-terminal stem segment of Influenza A HA subtype H11(no Cys-delta 1)
TKCQTEIGGINTNKSFHNVHRNTIGDCPKYVNVKSLKLATGPRNVPAIASR

SEQ ID NO: 258 - protein, 50 aa, Influenza virus A
  source 1..50: note = C-terminal stem segment of Influenza A HA subtype H11(no Cys-delta 3)
KCQTEIGGINTNKSFHNVHRNTIGDCPKYVNVKSLKLATGPRNVPAIASR

SEQ ID NO: 259 - protein, 52 aa, Influenza virus A
  source 1..52: note = C-terminal stem segment of Influenza A HA subtype H12(no Cys)
VTECQLNEGVMNTSKPFQNTSKHYIGKCPKYIPSGSLKLAIGLRNVPQVQDR

SEQ ID NO: 260 - protein, 51 aa, Influenza virus A
  source 1..51: note = C-terminal stem segment of Influenza A HA subtype H12(no Cys-delta 1)
TECQLNEGVMNTSKPFQNTSKHYIGKCPKYIPSGSLKLAIGLRNVPQVQDR

SEQ ID NO: 261 - protein, 50 aa, Influenza virus A
  source 1..50: note = C-terminal stem segment of Influenza A HA subtype H12(no Cys-delta 3)
ECQLNEGVMNTSKPFQNTSKHYIGKCPKYIPSGSLKLAIGLRNVPQVQDR

SEQ ID NO: 262 - protein, 52 aa, Influenza virus A
  source 1..52: note = C-terminal stem segment of Influenza A HA subtype H13(no Cys)
NTKCQTSVGGINTNRTFQNIDKNALGDCPKYIKSGQLKLATGLRNVPAISNR

SEQ ID NO: 263 - protein, 51 aa, Influenza virus A
  source 1..51: note = C-terminal stem segment of Influenza A HA subtype H13(no Cys-delta 1)
TKCQTSVGGINTNRTFQNIDKNALGDCPKYIKSGQLKLATGLRNVPAISNR

SEQ ID NO: 264 - protein, 50 aa, Influenza virus A
  source 1..50: note = C-terminal stem segment of Influenza A HA subtype H13(no Cys-delta 3)
KCQTSVGGINTNRTFQNIDKNALGDCPKYIKSGQLKLATGLRNVPAISNR

SEQ ID NO: 265 - protein, 52 aa, Influenza virus A
  source 1..52: note = C-terminal stem segment of Influenza A HA subtype H14(no Cys)
TSPCLTDKGSIQSDKPFQNVSRIAIGNCPKYVKQGSLMLATGMRNIPGKQAK

SEQ ID NO: 266 - protein, 51 aa, Influenza virus A
  source 1..51: note = C-terminal stem segment of Influenza A HA subtype H14(no Cys-delta 1)
SPCLTDKGSIQSDKPFQNVSRIAIGNCPKYVKQGSLMLATGMRNIPGKQAK

SEQ ID NO: 267 - protein, 50 aa, Influenza virus A
  source 1..50: note = C-terminal stem segment of Influenza A HA subtype H14(no Cys-delta 3)
PCLTDKGSIQSDKPFQNVSRIAIGNCPKYVKQGSLMLATGMRNIPGKQAK

SEQ ID NO: 268 - protein, 53 aa, Influenza virus A
  source 1..53: note = C-terminal stem segment of Influenza A HA subtype H15(no Cys)
EGECFYSGGTINSPLPFQNIDSRAVGKCPRYVKQSSLPLALGMKNVPEKIRTR

SEQ ID NO: 269 - protein, 52 aa, Influenza virus A
  source 1..52: note = C-terminal stem segment of Influenza A HA subtype H15(no Cys-delta 1)
GECFYSGGTINSPLPFQNIDSRAVGKCPRYVKQSSLPLALGMKNVPEKIRTR

SEQ ID NO: 270 - protein, 51 aa, Influenza virus A
  source 1..51: note = C-terminal stem segment of Influenza A HA subtype H15(no Cys-delta 3)
ECFYSGGTINSPLPFQNIDSRAVGKCPRYVKQSSLPLALGMKNVPEKIRTR

SEQ ID NO: 271 - protein, 52 aa, Influenza virus A
  source 1..52: note = C-terminal stem segment of Influenza A HA subtype H16(no Cys)
NTKCQTSLGGINTNKTFQNIERNALGDCPKYIKSGQLKLATGLRNVPSIGER

SEQ ID NO: 272 - protein, 51 aa, Influenza virus A
  source 1..51: note = C-terminal stem segment of Influenza A HA subtype H16(no Cys-delta 1)
TKCQTSLGGINTNKTFQNIERNALGDCPKYIKSGQLKLATGLRNVPSIGER

SEQ ID NO: 273 - protein, 50 aa, Influenza virus A
  source 1..50: note = C-terminal stem segment of Influenza A HA subtype H16(no Cys-delta 3)
KCQTSLGGINTNKTFQNIERNALGDCPKYIKSGQLKLATGLRNVPSIGER

SEQ ID NO: 274-307 - skipped (34 entries)

SEQ ID NO: 308 - protein, 44 aa, Influenza virus A
  source 1..44: note = N-terminal stem segment of Influenza A HA subtype H3(HK68-CON-A)
STATLCLGHHAVPNGTLVKTITDDQIEVTNATELVQSSSTGKIC

SEQ ID NO: 309 - protein, 24 aa, Influenza virus A
  source 1..24: note = C-terminal stem segment of Influenza A HA subtype H3(HK68-CON-B)
CKYVKQNTLKLATGMRNVPEKQTR

SEQ ID NO: 310 - protein, 97 aa, Influenza virus A
  source 1..97: note = N-terminal stem segment of Influenza A HA subtype H3(HK68-CON-C)
QDLPGNDNSTATLCLGHHAVPNGTLVKTITDDQIEVTNATELVQSSSTGKICNNPHRILDGIDCTLIDALLGDPHCDVFQNETWDLFVERSKAFSNC

SEQ ID NO: 311 - protein, 74 aa, Influenza virus A
  source 1..74: note = C-terminal stem segment of Influenza A HA subtype H3(HK68-CON-C)
APRGYFKMRTGKSSIMSSDAPIDTCISECITPNGSIPNDKPFQNVNKITYGACPKYVKQNTLKLATGMRNVPEK

SEQ ID NO: 312 - protein, 46 aa, Influenza virus A
  source 1..46: note = N-terminal stem segment of Influenza A HA subtype H1(HK68-CON-A)
DTICIGYHANNSTDTVDTVLEKNVTVTHSVNLLEDSHNGKLCRLKC

SEQ ID NO: 313 - protein, 52 aa, Influenza virus A
  source 1..52: note = C-terminal stem segment of Influenza A HA subtype H1(HK68-CON-A)
CKCQTPLGAINSSLPYQNIHPVTIGECPKYVRSAKLRMVTGLRNNPSIQSRG

SEQ ID NO: 314 - protein, 23 aa, Influenza virus A
  source 1..23: note = C-terminal stem segment of Influenza A HA subtype H1(HK68-CON-B)
CVRSAKLRMVTGLRNNPSIQSRG

SEQ ID NO: 315 - protein, 94 aa, Influenza virus A
  source 1..94: note = N-terminal stem segment of Influenza A HA subtype H1(HK68-CON-C)
DTICIGYHANNSTDTVDTVLEKNVTVTHSVNLLEDSHNGKLCRLKGIAPLQLGKCNIAGWLLGNPECDPLLPVRSWSYIVETPNSENGICYPGC

SEQ ID NO: 316 - protein, 75 aa, Influenza virus A
  source 1..75: note = C-terminal stem segment of Influenza A HA subtype H1(HK68-CON-C)
AFALSRGFGSGIITSNASMHECNTKCQTPLGAINSSLPYQNIHPVTIGECPKYVRSAKLRMVTGLRNNPSIQSRG

SEQ ID NO: 317-349 - skipped (33 entries)

SEQ ID NO: 350 - protein, 25 aa, Influenza virus A
  source 1..25: note = C-terminal short stem segment of Influenza A HA subtype H1
CPKYVRSAKLRMVTGLRNNPSIQSR

SEQ ID NO: 351 - protein, 25 aa, Influenza virus A
  source 1..25: note = C-terminal short stem segment of Influenza A HA subtype H2
CPKYVKSERLVLATGLRNVPQIESR

SEQ ID NO: 352 - protein, 25 aa, Influenza virus A
  source 1..25: note = C-terminal short stem segment of Influenza A HA subtype H3
CPKYVKQNTLKLATGMRNVPEKQTR

SEQ ID NO: 353 - protein, 25 aa, Influenza virus A
  source 1..25: note = C-terminal short stem segment of Influenza A HA subtype H4
CPRYVKQGSLKLATGMRNIPEKASR

SEQ ID NO: 354 - protein, 25 aa, Influenza virus A
  source 1..25: note = C-terminal short stem segment of Influenza A HA subtype H5
CPKYVKSDRLVLATGLRNVPQRKKR

SEQ ID NO: 355 - protein, 25 aa, Influenza virus A
  source 1..25: note = C-terminal short stem segment of Influenza A HA subtype H6
CPKYVKSESLRLATGLRNVPQIETR

SEQ ID NO: 356 - protein, 29 aa, Influenza virus A
  source 1..29: note = C-terminal short stem segment of Influenza A HA subtype H7
CPRYVKQESLLLATGMKNVPEPSKKRKKR

SEQ ID NO: 357 - protein, 25 aa, Influenza virus A
  source 1..25: note = C-terminal short stem segment of Influenza A HA subtype H8
CPKYVKKASLRLAVGLRNTPSVEPR

SEQ ID NO: 358 - protein, 25 aa, Influenza virus A
  source 1..25: note = C-terminal short stem segment of Influenza A HA subtype H9
CPKYVGVKSLKLPVGLRNVPAVSSR

SEQ ID NO: 359 - protein, 26 aa, Influenza virus A
  source 1..26: note = C-terminal short stem segment of Influenza A HA subtype H10
CPKYVNQRSLLLATGMRNVPEVVQGR

SEQ ID NO: 360 - protein, 25 aa, Influenza virus A
  source 1..25: note = C-terminal short stem segment of Influenza A HA subtype H11
CPKYVNVKSLKLATGPRNVPAIASR

SEQ ID NO: 361 - protein, 25 aa, Influenza virus A
  source 1..25: note = C-terminal short stem segment of Influenza A HA subtype H12
CPKYIPSGSLKLAIGLRNVPQVQDR

SEQ ID NO: 362 - protein, 25 aa, Influenza virus A
  source 1..25: note = C-terminal short stem segment of Influenza A HA subtype H13
CPKYIKSGQLKLATGLRNVPAISNR

SEQ ID NO: 363 - protein, 25 aa, Influenza virus A
  source 1..25: note = C-terminal short stem segment of Influenza A HA subtype H14
CPKYVKQGSLMLATGMRNIPGKQAK

SEQ ID NO: 364 - protein, 26 aa, Influenza virus A
  source 1..26: note = C-terminal short stem segment of Influenza A HA subtype H15
CPRYVKQSSLPLALGMKNVPEKIRTR

SEQ ID NO: 365 - protein, 25 aa, Influenza virus A
  source 1..25: note = C-terminal short stem segment of Influenza A HA subtype H16
CPKYIKSGQLKLATGLRNVPSIGER

SEQ ID NO: 366 - protein, 24 aa, Influenza virus A
  source 1..24: note = C-terminal stem segment of Influenza A HA subtype H1(no Cys)
PKYVRSAKLRMVTGLRNNPSIQSR

SEQ ID NO: 367 - protein, 23 aa, Influenza virus A
  source 1..23: note = C-terminal stem segment of Influenza A HA subtype H1(no Cys-delta 1)
KYVRSAKLRMVTGLRNNPSIQSR

SEQ ID NO: 368 - protein, 22 aa, Influenza virus A
  source 1..22: note = C-terminal stem segment of Influenza A HA subtype H1(no Cys-delta 3)
YVRSAKLRMVTGLRNNPSIQSR

SEQ ID NO: 369 - protein, 24 aa, Influenza virus A
  source 1..24: note = C-terminal stem segment of Influenza A HA subtype H2(no Cys)
PKYVKSERLVLATGLRNVPQIESR

SEQ ID NO: 370 - protein, 23 aa, Influenza virus A
  source 1..23: note = C-terminal stem segment of Influenza A HA subtype H2(no Cys-delta 1)
KYVKSERLVLATGLRNVPQIESR

SEQ ID NO: 371 - protein, 22 aa, Influenza virus A
  source 1..22: note = C-terminal stem segment of Influenza A HA subtype H2(no Cys-delta 3)
YVKSERLVLATGLRNVPQIESR

SEQ ID NO: 372 - protein, 24 aa, Influenza virus A
  source 1..24: note = C-terminal stem segment of Influenza A HA subtype H3(no Cys)
PKYVKQNTLKLATGMRNVPEKQTR

SEQ ID NO: 373 - protein, 23 aa, Influenza virus A
  source 1..23: note = C-terminal stem segment of Influenza A HA subtype H3(no Cys-delta 1)
KYVKQNTLKLATGMRNVPEKQTR

SEQ ID NO: 374 - protein, 22 aa, Influenza virus A
  source 1..22: note = C-terminal stem segment of Influenza A HA subtype H3(no Cys-delta 3)
YVKQNTLKLATGMRNVPEKQTR

SEQ ID NO: 375 - protein, 24 aa, Influenza virus A
  source 1..24: note = C-terminal stem segment of Influenza A HA subtype H4(no Cys)
PRYVKQGSLKLATGMRNIPEKASR

SEQ ID NO: 376 - protein, 23 aa, Influenza virus A
  source 1..23: note = C-terminal stem segment of Influenza A HA subtype H4(no Cys-delta 1)
RYVKQGSLKLATGMRNIPEKASR

SEQ ID NO: 377 - protein, 22 aa, Influenza virus A
  source 1..22: note = C-terminal stem segment of Influenza A HA subtype H4(no Cys-delta 3)
YVKQGSLKLATGMRNIPEKASR

SEQ ID NO: 378 - protein, 24 aa, Influenza virus A
  source 1..24: note = C-terminal stem segment of Influenza A HA subtype H5(no Cys)
PKYVKSDRLVLATGLRNVPQRKKR

SEQ ID NO: 379 - protein, 23 aa, Influenza virus A
  source 1..23: note = C-terminal stem segment of Influenza A HA subtype H5(no Cys-delta 1)
KYVKSDRLVLATGLRNVPQRKKR

SEQ ID NO: 380 - protein, 22 aa, Influenza virus A
  source 1..22: note = C-terminal stem segment of Influenza A HA subtype H5(no Cys-delta 3)
YVKSDRLVLATGLRNVPQRKKR

SEQ ID NO: 381 - protein, 24 aa, Influenza virus A
  source 1..24: note = C-terminal stem segment of Influenza A HA subtype H6(no Cys)
PKYVKSESLRLATGLRNVPQIETR

SEQ ID NO: 382 - protein, 23 aa, Influenza virus A
  source 1..23: note = C-terminal stem segment of Influenza A HA subtype H6(no Cys-delta 1)
KYVKSESLRLATGLRNVPQIETR

SEQ ID NO: 383 - protein, 22 aa, Influenza virus A
  source 1..22: note = C-terminal stem segment of Influenza A HA subtype H6(no Cys-delta 3)
YVKSESLRLATGLRNVPQIETR

SEQ ID NO: 384 - protein, 28 aa, Influenza virus A
  source 1..28: note = C-terminal stem segment of Influenza A HA subtype H7(no Cys)
PRYVKQESLLLATGMKNVPEPSKKRKKR

SEQ ID NO: 385 - protein, 27 aa, Influenza virus A
  source 1..27: note = C-terminal stem segment of Influenza A HA subtype H7(no Cys-delta 1)
RYVKQESLLLATGMKNVPEPSKKRKKR

SEQ ID NO: 386 - protein, 26 aa, Influenza virus A
  source 1..26: note = C-terminal stem segment of Influenza A HA subtype H7(no Cys-delta 3)
YVKQESLLLATGMKNVPEPSKKRKKR

SEQ ID NO: 387 - protein, 24 aa, Influenza virus A
  source 1..24: note = C-terminal stem segment of Influenza A HA subtype H8(no Cys)
PKYVKKASLRLAVGLRNTPSVEPR

SEQ ID NO: 388 - protein, 23 aa, Influenza virus A
  source 1..23: note = C-terminal stem segment of Influenza A HA subtype H8(no Cys-delta 1)
KYVKKASLRLAVGLRNTPSVEPR

SEQ ID NO: 389 - protein, 22 aa, Influenza virus A
  source 1..22: note = C-terminal stem segment of Influenza A HA subtype H8(no Cys-delta 3)
YVKKASLRLAVGLRNTPSVEPR

SEQ ID NO: 390 - protein, 24 aa, Influenza virus A
  source 1..24: note = C-terminal stem segment of Influenza A HA subtype H9(no Cys)
PKYVGVKSLKLPVGLRNVPAVSSR

SEQ ID NO: 391 - protein, 23 aa, Influenza virus A
  source 1..23: note = C-terminal stem segment of Influenza A HA subtype H9(no Cys-delta 1)
KYVGVKSLKLPVGLRNVPAVSSR

SEQ ID NO: 392 - protein, 22 aa, Influenza virus A
  source 1..22: note = C-terminal stem segment of Influenza A HA subtype H9(no Cys-delta 3)
YVGVKSLKLPVGLRNVPAVSSR

SEQ ID NO: 393 - protein, 25 aa, Influenza virus A
  source 1..25: note = C-terminal stem segment of Influenza A HA subtype H10(no Cys)
PKYVNQRSLLLATGMRNVPEVVQGR

SEQ ID NO: 394 - protein, 24 aa, Influenza virus A
  source 1..24: note = C-terminal stem segment of Influenza A HA subtype H10(no Cys-delta 1)
KYVNQRSLLLATGMRNVPEVVQGR

SEQ ID NO: 395 - protein, 23 aa, Influenza virus A
  source 1..23: note = C-terminal stem segment of Influenza A HA subtype H10(no Cys-delta 3)
YVNQRSLLLATGMRNVPEVVQGR

SEQ ID NO: 396 - protein, 24 aa, Influenza virus A
  source 1..24: note = C-terminal stem segment of Influenza A HA subtype H11(no Cys)
PKYVNVKSLKLATGPRNVPAIASR

SEQ ID NO: 397 - protein, 23 aa, Influenza virus A
  source 1..23: note = C-terminal stem segment of Influenza A HA subtype H11(no Cys-delta 1)
KYVNVKSLKLATGPRNVPAIASR

SEQ ID NO: 398 - protein, 22 aa, Influenza virus A
  source 1..22: note = C-terminal stem segment of Influenza A HA subtype H11(no Cys-delta 3)
YVNVKSLKLATGPRNVPAIASR

SEQ ID NO: 399 - protein, 24 aa, Influenza virus A
  source 1..24: note = C-terminal stem segment of Influenza A HA subtype H12(no Cys)
PKYIPSGSLKLAIGLRNVPQVQDR

SEQ ID NO: 400 - protein, 23 aa, Influenza virus A
  source 1..23: note = C-terminal stem segment of Influenza A HA subtype H12(no Cys-delta 1)
KYIPSGSLKLAIGLRNVPQVQDR

SEQ ID NO: 401 - protein, 22 aa, Influenza virus A
  source 1..22: note = C-terminal stem segment of Influenza A HA subtype H12(no Cys-delta 3)
YIPSGSLKLAIGLRNVPQVQDR

SEQ ID NO: 402 - protein, 24 aa, Influenza virus A
  source 1..24: note = C-terminal stem segment of Influenza A HA subtype H13(no Cys)
PKYIKSGQLKLATGLRNVPAISNR

SEQ ID NO: 403 - protein, 23 aa, Influenza virus A
  source 1..23: note = C-terminal stem segment of Influenza A HA subtype H13(no Cys-delta 1)
KYIKSGQLKLATGLRNVPAISNR

SEQ ID NO: 404 - protein, 22 aa, Influenza virus A
  source 1..22: note = C-terminal stem segment of Influenza A HA subtype H13(no Cys-delta 3)
YIKSGQLKLATGLRNVPAISNR

SEQ ID NO: 405 - protein, 24 aa, Influenza virus A
  source 1..24: note = C-terminal stem segment of Influenza A HA subtype H14(no Cys)
PKYVKQGSLMLATGMRNIPGKQAK

SEQ ID NO: 406 - protein, 23 aa, Influenza virus A
  source 1..23: note = C-terminal stem segment of Influenza A HA subtype H14(no Cys-delta 1)
KYVKQGSLMLATGMRNIPGKQAK

SEQ ID NO: 407 - protein, 22 aa, Influenza virus A
  source 1..22: note = C-terminal stem segment of Influenza A HA subtype H14(no Cys-delta 3)
YVKQGSLMLATGMRNIPGKQAK

SEQ ID NO: 408 - protein, 25 aa, Influenza virus A
  source 1..25: note = C-terminal stem segment of Influenza A HA subtype H15(no Cys)
PRYVKQSSLPLALGMKNVPEKIRTR

SEQ ID NO: 409 - protein, 24 aa, Influenza virus A
  source 1..24: note = C-terminal stem segment of Influenza A HA subtype H15(no Cys-delta 1)
RYVKQSSLPLALGMKNVPEKIRTR

SEQ ID NO: 410 - protein, 23 aa, Influenza virus A
  source 1..23: note = C-terminal stem segment of Influenza A HA subtype H15(no Cys-delta 3)
YVKQSSLPLALGMKNVPEKIRTR

SEQ ID NO: 411 - protein, 24 aa, Influenza virus A
  source 1..24: note = C-terminal stem segment of Influenza A HA subtype H16(no Cys)
PKYIKSGQLKLATGLRNVPSIGER

SEQ ID NO: 412 - protein, 23 aa, Influenza virus A
  source 1..23: note = C-terminal stem segment of Influenza A HA subtype H16(no Cys-delta 1)
KYIKSGQLKLATGLRNVPSIGER

SEQ ID NO: 413 - protein, 22 aa, Influenza virus A
  source 1..22: note = C-terminal stem segment of Influenza A HA subtype H16(no Cys-delta 3)
YIKSGQLKLATGLRNVPSIGER

SEQ ID NO: 414 - protein, 90 aa, Influenza virus A
  source 1..90: note = N-termianl long stem domain segment of Influenza A HA subtype H1
DTICIGYHANNSTDTVDTVLEKNVTVTHSVNLLEDSHNGKLCRLKGIAPLQLGKCNIAGWLLGNPECDPLLPVRSWSYIVETPNSENGIC

SEQ ID NO: 415 - protein, 90 aa, Influenza virus A
  source 1..90: note = N-termianl long stem domain segment of Influenza A HA subtype H2
DQICIGYHSNNSTEKVDTILERNVTVTHAQNILEKTHNGKLCKLNGIPPLELGDCSIAGWLLGNPECDRLLTVPEWSYIMEKENPRNGLC

SEQ ID NO: 416 - protein, 97 aa, Influenza virus A; identical to SEQ ID NO: 310
  source 1..97: note = N-termianl long stem domain segment of Influenza A HA subtype H3

SEQ ID NO: 417 - protein, 93 aa, Influenza virus A
  source 1..93: note = N-termianl long stem domain segment of Influenza A HA subtype H4
QNYTGNPVICMGHHAVANGTMVKTLADDQVEVVTAQELVESQNLPELCPSPLRLVDGQTCDIINGALGSPGCDHLNGAEWDVFIERPNAVDTC

SEQ ID NO: 418 - protein, 90 aa, Influenza virus A
  source 1..90: note = N-termianl long stem domain segment of Influenza A HA subtype H5
DQICIGYHANKSTKQVDTIMEKNVTVTHAQDILERTHNGKLCSLNGVKPLILRDCSVAGWLLGNPMCDEFLNLPEWLYIVEKDNPINSLC

SEQ ID NO: 419 - protein, 90 aa, Influenza virus A
  source 1..90: note = N-termianl long stem domain segment of Influenza A HA subtype H6
DKICIGYHANNSTTQIDTILEKNVTVTHSVELLENQKEERFCKILKKAPLDLKGCTIEGWILGNPQCDLLLGDQSWSYIVERPTAQNGIC

SEQ ID NO: 420 - protein, 87 aa, Influenza virus A
  source 1..87: note = N-termianl long stem domain segment of Influenza A HA subtype H7
DKICLGHHAVSNGTKVNTLTERGVEVVNATETVERTNIPKICSKGKRTTDLGQCGLLGTITGPPQCDQFLEFSADLIIERREGNDVC

SEQ ID NO: 421 - protein, 90 aa, Influenza virus A
  source 1..90: note = N-termianl long stem domain segment of Influenza A HA subtype H8
DRICIGYQSNNSTDTVNTLIEQNVPVTQTMELVETEKHPAYCNTDLGAPLELRDCKIEAVIYGNPKCDIHLKDQGWSYIVERPSAPEGMC

SEQ ID NO: 422 - protein, 90 aa, Influenza virus A
  source 1..90: note = N-termianl long stem domain segment of Influenza A HA subtype H9
DKICIGYQSTNSTETVDTLTESNVPVTHTKELLHTEHNGMLCATDLGHPLILDTCTIEGLIYGNPSCDILLGGKEWSYIVERSSAVNGMC

SEQ ID NO: 423 - protein, 88 aa, Influenza virus A
  source 1..88: note = N-termianl long stem domain segment of Influenza A HA subtype H10
LDRICLGHHAVANGTIVKTLTNEQEEVTNATETVESTNLNKLCMKGRSYKDLGNCHPVGMLIGTPVCDPHLTGTWDTLIERENAIAHC

SEQ ID NO: 424 - protein, 90 aa, Influenza virus A
  source 1..90: note = N-termianl long stem domain segment of Influenza A HA subtype H11
DEICIGYLSNNSTDKVDTIIENNVTVTSSVELVETEHTGSFCSINGKQPISLGDCSFAGWILGNPMCDELIGKTSWSYIVEKPNPTNGIC

SEQ ID NO: 425 - protein, 90 aa, Influenza virus A
  source 1..90: note = N-termianl long stem domain segment of Influenza A HA subtype H12
DKICIGYQTNNSTETVNTLSEQNVPVTQVEELVHRGIDPILCGTELGSPLVLDDCSLEGLILGNPKCDLYLNGREWSYIVERPKEMEGVC

SEQ ID NO: 426 - protein, 90 aa, Influenza virus A
  source 1..90: note = N-termianl long stem domain segment of Influenza A HA subtype H13
DRICVGYLSTNSSERVDTLLENGVPVTSSIDLIETNHTGTYCSLNGVSPVHLGDCSFEGWIVGNPACTSNFGIREWSYLIEDPAAPHGLC

SEQ ID NO: 427 - protein, 96 aa, Influenza virus A
  source 1..96: note = N-termianl long stem domain segment of Influenza A HA subtype H14
QITNGTTGNPIICLGHHAVENGTSVKTLTDNHVEVVSAKELVETNHTDELCPSPLKLVDGQDCHLINGALGSPGCDRLQDTTWDVFIERPTAVDTC

SEQ ID NO: 428 - protein, 87 aa, Influenza virus A
  source 1..87: note = N-termianl long stem domain segment of Influenza A HA subtype H15
DKICLGHHAVANGTKVNTLTERGVEVVNATETVEITGIDKVCTKGKKAVDLGSCGILGTIIGPPQCDLHLEFKADLIIERRNSSDIC

SEQ ID NO: 429 - protein, 90 aa, Influenza virus A
  source 1..90: note = N-termianl long stem domain segment of Influenza A HA subtype H16
DKICIGYLSNNSSDTVDTLTENGVPVTSSVDLVETNHTGTYCSLNGISPIHLGDCSFEGWIVGNPSCATNINIREWSYLIEDPNAPNKFC

SEQ ID NO: 430 - protein, 78 aa, Influenza virus A
  source 1..78: note = C-termianl long stem domain segment of Influenza A HA subtype H1
APMYAFALSRGFGSGIITSNASMHECNTKCQTPLGAINSSLPYQNIHPVTIGECPKYVRSAKLRMVTGLRNNPSIQSR

SEQ ID NO: 431 - protein, 78 aa, Influenza virus A
  source 1..78: note = C-termianl long stem domain segment of Influenza A HA subtype H2
APEYGFRISKRGSSGIMKTEGTLENCETKCQTPLGAINTTLPFHNVHPLTIGECPKYVKSERLVLATGLRNVPQIESR

SEQ ID NO: 432 - protein, 77 aa, Influenza virus A
  source 1..77: note = C-termianl long stem domain segment of Influenza A HA subtype H3
APRGYFKMRTGKSSIMSSDAPIDTCISECITPNGSIPNDKPFQNVNKITYGACPKYVKQNTLKLATGMRNVPEKQTR

SEQ ID NO: 433 - protein, 78 aa, Influenza virus A
  source 1..78: note = C-termianl long stem domain segment of Influenza A HA subtype H4
APRGHYKLNNQKKSTILNTAIPIGSCVSKCHTDKGSLSTTKPFQNISRIAVGDCPRYVKQGSLKLATGMRNIPEKASR

SEQ ID NO: 434 - protein, 78 aa, Influenza virus A
  source 1..78: note = C-termianl long stem domain segment of Influenza A HA subtype H5
APRYAYKIVKKGDSAIMKSGLAYGNCDTKCQTPVGEINSSMPFHNIHPHTIGECPKYVKSDRLVLATGLRNVPQRKKR

SEQ ID NO: 435 - protein, 79 aa, Influenza virus A
  source 1..79: note = C-termianl long stem domain segment of Influenza A HA subtype H6
APWYAFRFVSTSNKGAVFKSNLPIENCDATCQTVAGVLRTNKTFQNVSPLWIGECPKYVKSESLRLATGLRNVPQIETR

SEQ ID NO: 436 - protein, 81 aa, Influenza virus A
  source 1..81: note = C-termianl long stem domain segment of Influenza A HA subtype H7
APNRASFLRGKSMGIQSDVQVDANCEGECYHSGGTITSRLPFQNINSRAVGKCPRYVKQESLLLATGMKNVPEPSKKRKKR

SEQ ID NO: 437 - protein, 79 aa, Influenza virus A
  source 1..79: note = C-termianl long stem domain segment of Influenza A HA subtype H8
APEFGYLLKGESYGRIIQNEDIPIGNCNTKCQTYAGAINSSKPFQNASRHYMGECPKYVKKASLRLAVGLRNTPSVEPR

SEQ ID NO: 438 - protein, 78 aa, Influenza virus A
  source 1..78: note = C-termianl long stem domain segment of Influenza A HA subtype H9
APWYGHVLTGESHGRILKTDLNNGNCVVQCQTEKGGLNTTLPFHNISKYAFGNCPKYVGVKSLKLPVGLRNVPAVSSR

SEQ ID NO: 439 - protein, 78 aa, Influenza virus A
  source 1..78: note = C-termianl long stem domain segment of Influenza A HA subtype H10
APSRVSKLTGRDLGIQSEALIDNSCESKCFWRGGSINTKLPFQNLSPRTVGQCPKYVNQRSLLLATGMRNVPEVVQGR

SEQ ID NO: 440 - protein, 78 aa, Influenza virus A
  source 1..78: note = C-termianl long stem domain segment of Influenza A HA subtype H11
APRYAFEIVSVGNGKLFRSELNIESCSTKCQTEIGGINTNKSFHNVHRNTIGDCPKYVNVKSLKLATGPRNVPAIASR

SEQ ID NO: 441 - protein, 78 aa, Influenza virus A
  source 1..78: note = C-termianl long stem domain segment of Influenza A HA subtype H12
APEYGHLITGKSHGRILKNNLPMGQCVTECQLNEGVMNTSKPFQNTSKHYIGKCPKYIPSGSLKLAIGLRNVPQVQDR

SEQ ID NO: 442 - protein, 78 aa, Influenza virus A
  source 1..78: note = C-termianl long stem domain segment of Influenza A HA subtype H13
APRYGYIIEEYGKGRIFQSRIRMSRCNTKCQTSVGGINTNRTFQNIDKNALGDCPKYIKSGQLKLATGLRNVPAISNR

SEQ ID NO: 443 - protein, 78 aa, Influenza virus A
  source 1..78: note = C-termianl long stem domain segment of Influenza A HA subtype H14
APRGHYKISKSTKSTVLKSDKRIGSCTSPCLTDKGSIQSDKPFQNVSRIAIGNCPKYVKQGSLMLATGMRNIPGKQAK

SEQ ID NO: 444 - protein, 88 aa, Influenza virus A
  source 1..88: note = C-termianl long stem domain segment of Influenza A HA subtype H15
APDRATFLRSNAPSGIEYNGKSLGIQSDAQIDESCEGECFYSGGTINSPLPFQNIDSRAVGKCPRYVKQSSLPLALGMKNVPEKIRTR

SEQ ID NO: 445 - protein, 78 aa, Influenza virus A
  source 1..78: note = C-termianl long stem domain segment of Influenza A HA subtype H16
APRYGYIIEKYGTGRIFQSGVRMARCNTKCQTSLGGINTNKTFQNIERNALGDCPKYIKSGQLKLATGLRNVPSIGER

SEQ ID NO: 446 - protein, 89 aa, Influenza virus A
  source 1..89: note = N-termianl long stem domain segment of Influenza A HA subtype H1(No Cys, Ala)
DTICIGYHANNSTDTVDTVLEKNVTVTHSVNLLEDSHNGKLCRLKGIAPLQLGKCNIAGWLLGNPECDPLLPVRSWSYIVETPNSENGI

SEQ ID NO: 447 - protein, 89 aa, Influenza virus A; identical to SEQ ID NO: 446
  source 1..89: note = N-termianl long stem domain segment of Influenza A HA subtype H1(No Cys, Ala - Delta 1)

SEQ ID NO: 448 - protein, 88 aa, Influenza virus A
  source 1..88: note = N-termianl long stem domain segment of Influenza A HA subtype H1(No Cys, Ala - Delta 3)
DTICIGYHANNSTDTVDTVLEKNVTVTHSVNLLEDSHNGKLCRLKGIAPLQLGKCNIAGWLLGNPECDPLLPVRSWSYIVETPNSENG

SEQ ID NO: 449 - protein, 89 aa, Influenza virus A
  source 1..89: note = N-termianl long stem domain segment of Influenza A HA subtype H2(No Cys, Ala)
DQICIGYHSNNSTEKVDTILERNVTVTHAQNILEKTHNGKLCKLNGIPPLELGDCSIAGWLLGNPECDRLLTVPEWSYIMEKENPRNGL

SEQ ID NO: 450 - protein, 89 aa, Influenza virus A; identical to SEQ ID NO: 449
  source 1..89: note = N-termianl long stem domain segment of Influenza A HA subtype H2(No Cys, Ala - Delta 1)

SEQ ID NO: 451 - protein, 88 aa, Influenza virus A
  source 1..88: note = N-termianl long stem domain segment of Influenza A HA subtype H2(No Cys, Ala - Delta 3)
DQICIGYHSNNSTEKVDTILERNVTVTHAQNILEKTHNGKLCKLNGIPPLELGDCSIAGWLLGNPECDRLLTVPEWSYIMEKENPRNG

SEQ ID NO: 452 - protein, 96 aa, Influenza virus A
  source 1..96: note = N-termianl long stem domain segment of Influenza A HA subtype H3(No Cys, Ala)
QDLPGNDNSTATLCLGHHAVPNGTLVKTITDDQIEVTNATELVQSSSTGKICNNPHRILDGIDCTLIDALLGDPHCDVFQNETWDLFVERSKAFSN

SEQ ID NO: 453 - protein, 96 aa, Influenza virus A; identical to SEQ ID NO: 452
  source 1..96: note = N-termianl long stem domain segment of Influenza A HA subtype H3(No Cys, Ala - Delta 1)

SEQ ID NO: 454 - protein, 95 aa, Influenza virus A
  source 1..95: note = N-termianl long stem domain segment of Influenza A HA subtype H3(No Cys, Ala - Delta 3)
QDLPGNDNSTATLCLGHHAVPNGTLVKTITDDQIEVTNATELVQSSSTGKICNNPHRILDGIDCTLIDALLGDPHCDVFQNETWDLFVERSKAFS

SEQ ID NO: 455 - protein, 92 aa, Influenza virus A
  source 1..92: note = N-termianl long stem domain segment of Influenza A HA subtype H4(No Cys, Ala)
QNYTGNPVICMGHHAVANGTMVKTLADDQVEVVTAQELVESQNLPELCPSPLRLVDGQTCDIINGALGSPGCDHLNGAEWDVFIERPNAVDT

SEQ ID NO: 456 - protein, 92 aa, Influenza virus A; identical to SEQ ID NO: 455
  source 1..92: note = N-termianl long stem domain segment of Influenza A HA subtype H4(No Cys, Ala - Delta 1)

SEQ ID NO: 457 - protein, 91 aa, Influenza virus A
  source 1..91: note = N-termianl long stem domain segment of Influenza A HA subtype H4(No Cys, Ala - Delta 3)
QNYTGNPVICMGHHAVANGTMVKTLADDQVEVVTAQELVESQNLPELCPSPLRLVDGQTCDIINGALGSPGCDHLNGAEWDVFIERPNAVD

SEQ ID NO: 458 - protein, 89 aa, Influenza virus A
  source 1..89: note = N-termianl long stem domain segment of Influenza A HA subtype H5(No Cys, Ala)
DQICIGYHANKSTKQVDTIMEKNVTVTHAQDILERTHNGKLCSLNGVKPLILRDCSVAGWLLGNPMCDEFLNLPEWLYIVEKDNPINSL

SEQ ID NO: 459 - protein, 89 aa, Influenza virus A; identical to SEQ ID NO: 458
  source 1..89: note = N-termianl long stem domain segment of Influenza A HA subtype H5(No Cys, Ala - Delta 1)

SEQ ID NO: 460 - protein, 88 aa, Influenza virus A
  source 1..88: note = N-termianl long stem domain segment of Influenza A HA subtype H5(No Cys, Ala - Delta 3)
DQICIGYHANKSTKQVDTIMEKNVTVTHAQDILERTHNGKLCSLNGVKPLILRDCSVAGWLLGNPMCDEFLNLPEWLYIVEKDNPINS

SEQ ID NO: 461 - protein, 89 aa, Influenza virus A
  source 1..89: note = N-termianl long stem domain segment of Influenza A HA subtype H6(No Cys, Ala)
DKICIGYHANNSTTQIDTILEKNVTVTHSVELLENQKEERFCKILKKAPLDLKGCTIEGWILGNPQCDLLLGDQSWSYIVERPTAQNGI

SEQ ID NO: 462 - protein, 89 aa, Influenza virus A; identical to SEQ ID NO: 461
  source 1..89: note = N-termianl long stem domain segment of Influenza A HA subtype H6(No Cys, Ala - Delta 1)

SEQ ID NO: 463 - protein, 88 aa, Influenza virus A
  source 1..88: note = N-termianl long stem domain segment of Influenza A HA subtype H6(No Cys, Ala - Delta 3)
DKICIGYHANNSTTQIDTILEKNVTVTHSVELLENQKEERFCKILKKAPLDLKGCTIEGWILGNPQCDLLLGDQSWSYIVERPTAQNG

SEQ ID NO: 464 - protein, 86 aa, Influenza virus A
  source 1..86: note = N-termianl long stem domain segment of Influenza A HA subtype H7(No Cys, Ala)
DKICLGHHAVSNGTKVNTLTERGVEVVNATETVERTNIPKICSKGKRTTDLGQCGLLGTITGPPQCDQFLEFSADLIIERREGNDV

SEQ ID NO: 465 - protein, 86 aa, Influenza virus A; identical to SEQ ID NO: 464
  source 1..86: note = N-termianl long stem domain segment of Influenza A HA subtype H7(No Cys, Ala - Delta 1)

SEQ ID NO: 466 - protein, 85 aa, Influenza virus A
  source 1..85: note = N-termianl long stem domain segment of Influenza A HA subtype H7(No Cys, Ala - Delta 3)
DKICLGHHAVSNGTKVNTLTERGVEVVNATETVERTNIPKICSKGKRTTDLGQCGLLGTITGPPQCDQFLEFSADLIIERREGND

SEQ ID NO: 467 - protein, 89 aa, Influenza virus A
  source 1..89: note = N-termianl long stem domain segment of Influenza A HA subtype H8(No Cys, Ala)
DRICIGYQSNNSTDTVNTLIEQNVPVTQTMELVETEKHPAYCNTDLGAPLELRDCKIEAVIYGNPKCDIHLKDQGWSYIVERPSAPEGM

SEQ ID NO: 468 - protein, 89 aa, Influenza virus A; identical to SEQ ID NO: 467
  source 1..89: note = N-termianl long stem domain segment of Influenza A HA subtype H8(No Cys, Ala - Delta 1)

SEQ ID NO: 469 - protein, 88 aa, Influenza virus A
  source 1..88: note = N-termianl long stem domain segment of Influenza A HA subtype H8(No Cys, Ala - Delta 3)
DRICIGYQSNNSTDTVNTLIEQNVPVTQTMELVETEKHPAYCNTDLGAPLELRDCKIEAVIYGNPKCDIHLKDQGWSYIVERPSAPEG

SEQ ID NO: 470 - protein, 89 aa, Influenza virus A
  source 1..89: note = N-termianl long stem domain segment of Influenza A HA subtype H9(No Cys, Ala)
DKICIGYQSTNSTETVDTLTESNVPVTHTKELLHTEHNGMLCATDLGHPLILDTCTIEGLIYGNPSCDILLGGKEWSYIVERSSAVNGM

SEQ ID NO: 471 - protein, 89 aa, Influenza virus A; identical to SEQ ID NO: 470
  source 1..89: note = N-termianl long stem domain segment of Influenza A HA subtype H9(No Cys, Ala - Delta 1)

SEQ ID NO: 472 - protein, 88 aa, Influenza virus A
  source 1..88: note = N-termianl long stem domain segment of Influenza A HA subtype H9(No Cys, Ala - Delta 3)
DKICIGYQSTNSTETVDTLTESNVPVTHTKELLHTEHNGMLCATDLGHPLILDTCTIEGLIYGNPSCDILLGGKEWSYIVERSSAVNG

SEQ ID NO: 473 - protein, 87 aa, Influenza virus A
  source 1..87: note = N-termianl long stem domain segment of Influenza A HA subtype H10(No Cys, Ala)
LDRICLGHHAVANGTIVKTLTNEQEEVTNATETVESTNLNKLCMKGRSYKDLGNCHPVGMLIGTPVCDPHLTGTWDTLIERENAIAH

SEQ ID NO: 474 - protein, 87 aa, Influenza virus A; identical to SEQ ID NO: 473
  source 1..87: note = N-termianl long stem domain segment of Influenza A HA subtype H10(No Cys, Ala - Delta 1)

SEQ ID NO: 475 - protein, 86 aa, Influenza virus A
  source 1..86: note = N-termianl long stem domain segment of Influenza A HA subtype H10(No Cys, Ala - Delta 3)
LDRICLGHHAVANGTIVKTLTNEQEEVTNATETVESTNLNKLCMKGRSYKDLGNCHPVGMLIGTPVCDPHLTGTWDTLIERENAIA

SEQ ID NO: 476 - protein, 89 aa, Influenza virus A
  source 1..89: note = N-termianl long stem domain segment of Influenza A HA subtype H11(No Cys, Ala)
DEICIGYLSNNSTDKVDTIIENNVTVTSSVELVETEHTGSFCSINGKQPISLGDCSFAGWILGNPMCDELIGKTSWSYIVEKPNPTNGI

SEQ ID NO: 477 - protein, 89 aa, Influenza virus A; identical to SEQ ID NO: 476
  source 1..89: note = N-termianl long stem domain segment of Influenza A HA subtype H11(No Cys, Ala - Delta 1)

SEQ ID NO: 478 - protein, 88 aa, Influenza virus A
  source 1..88: note = N-termianl long stem domain segment of Influenza A HA subtype H11(No Cys, Ala - Delta 3)
DEICIGYLSNNSTDKVDTIIENNVTVTSSVELVETEHTGSFCSINGKQPISLGDCSFAGWILGNPMCDELIGKTSWSYIVEKPNPTNG

SEQ ID NO: 479 - protein, 89 aa, Influenza virus A
  source 1..89: note = N-termianl long stem domain segment of Influenza A HA subtype H12(No Cys, Ala)
DKICIGYQTNNSTETVNTLSEQNVPVTQVEELVHRGIDPILCGTELGSPLVLDDCSLEGLILGNPKCDLYLNGREWSYIVERPKEMEGV

SEQ ID NO: 480 - protein, 89 aa, Influenza virus A; identical to SEQ ID NO: 479
  source 1..89: note = N-termianl long stem domain segment of Influenza A HA subtype H12(No Cys, Ala - Delta 1)

SEQ ID NO: 481 - protein, 88 aa, Influenza virus A
  source 1..88: note = N-termianl long stem domain segment of Influenza A HA subtype H12(No Cys, Ala - Delta 3)
DKICIGYQTNNSTETVNTLSEQNVPVTQVEELVHRGIDPILCGTELGSPLVLDDCSLEGLILGNPKCDLYLNGREWSYIVERPKEMEG

SEQ ID NO: 482 - protein, 89 aa, Influenza virus A
  source 1..89: note = N-termianl long stem domain segment of Influenza A HA subtype H13(No Cys, Ala)
DRICVGYLSTNSSERVDTLLENGVPVTSSIDLIETNHTGTYCSLNGVSPVHLGDCSFEGWIVGNPACTSNFGIREWSYLIEDPAAPHGL

SEQ ID NO: 483 - protein, 89 aa, Influenza virus A; identical to SEQ ID NO: 482
  source 1..89: note = N-termianl long stem domain segment of Influenza A HA subtype H13(No Cys, Ala - Delta 1)

SEQ ID NO: 484 - protein, 88 aa, Influenza virus A
  source 1..88: note = N-termianl long stem domain segment of Influenza A HA subtype H13(No Cys, Ala - Delta 3)
DRICVGYLSTNSSERVDTLLENGVPVTSSIDLIETNHTGTYCSLNGVSPVHLGDCSFEGWIVGNPACTSNFGIREWSYLIEDPAAPHG

SEQ ID NO: 485 - protein, 95 aa, Influenza virus A
  source 1..95: note = N-termianl long stem domain segment of Influenza A HA subtype H14(No Cys, Ala)
QITNGTTGNPIICLGHHAVENGTSVKTLTDNHVEVVSAKELVETNHTDELCPSPLKLVDGQDCHLINGALGSPGCDRLQDTTWDVFIERPTAVDT

SEQ ID NO: 486 - protein, 95 aa, Influenza virus A; identical to SEQ ID NO: 485
  source 1..95: note = N-termianl long stem domain segment of Influenza A HA subtype H14(No Cys, Ala - Delta 1)

SEQ ID NO: 487 - protein, 94 aa, Influenza virus A
  source 1..94: note = N-termianl long stem domain segment of Influenza A HA subtype H14(No Cys, Ala - Delta 3)
QITNGTTGNPIICLGHHAVENGTSVKTLTDNHVEVVSAKELVETNHTDELCPSPLKLVDGQDCHLINGALGSPGCDRLQDTTWDVFIERPTAVD

SEQ ID NO: 488 - protein, 86 aa, Influenza virus A
  source 1..86: note = N-termianl long stem domain segment of Influenza A HA subtype H15(No Cys, Ala)
DKICLGHHAVANGTKVNTLTERGVEVVNATETVEITGIDKVCTKGKKAVDLGSCGILGTIIGPPQCDLHLEFKADLIIERRNSSDI

SEQ ID NO: 489 - protein, 86 aa, Influenza virus A; identical to SEQ ID NO: 488
  source 1..86: note = N-termianl long stem domain segment of Influenza A HA subtype H15(No Cys, Ala - Delta 1)

SEQ ID NO: 490 - protein, 85 aa, Influenza virus A
  source 1..85: note = N-termianl long stem domain segment of Influenza A HA subtype H15(No Cys, Ala - Delta 3)
DKICLGHHAVANGTKVNTLTERGVEVVNATETVEITGIDKVCTKGKKAVDLGSCGILGTIIGPPQCDLHLEFKADLIIERRNSSD

SEQ ID NO: 491 - protein, 89 aa, Influenza virus A
  source 1..89: note = N-termianl long stem domain segment of Influenza A HA subtype H16(No Cys, Ala)
DKICIGYLSNNSSDTVDTLTENGVPVTSSVDLVETNHTGTYCSLNGISPIHLGDCSFEGWIVGNPSCATNINIREWSYLIEDPNAPNKF

SEQ ID NO: 492 - protein, 89 aa, Influenza virus A; identical to SEQ ID NO: 491
  source 1..89: note = N-termianl long stem domain segment of Influenza A HA subtype H16(No Cys, Ala - Delta 1)

SEQ ID NO: 493 - protein, 88 aa, Influenza virus A
  source 1..88: note = N-termianl long stem domain segment of Influenza A HA subtype H16(No Cys, Ala - Delta 3)
DKICIGYLSNNSSDTVDTLTENGVPVTSSVDLVETNHTGTYCSLNGISPIHLGDCSFEGWIVGNPSCATNINIREWSYLIEDPNAPNK

SEQ ID NO: 494 - protein, 77 aa, Influenza virus A
  source 1..77: note = C-termianl long stem domain segment of Influenza A HA subtype H1(No Cys, Ala)
PMYAFALSRGFGSGIITSNASMHECNTKCQTPLGAINSSLPYQNIHPVTIGECPKYVRSAKLRMVTGLRNNPSIQSR

SEQ ID NO: 495 - protein, 76 aa, Influenza virus A
  source 1..76: note = C-termianl long stem domain segment of Influenza A HA subtype H1(No Cys, Ala - Delta 1)
MYAFALSRGFGSGIITSNASMHECNTKCQTPLGAINSSLPYQNIHPVTIGECPKYVRSAKLRMVTGLRNNPSIQSR

SEQ ID NO: 496 - protein, 75 aa, Influenza virus A
  source 1..75: note = C-termianl long stem domain segment of Influenza A HA subtype H1(No Cys, Ala - Delta 3)
YAFALSRGFGSGIITSNASMHECNTKCQTPLGAINSSLPYQNIHPVTIGECPKYVRSAKLRMVTGLRNNPSIQSR

SEQ ID NO: 497 - protein, 77 aa, Influenza virus A
  source 1..77: note = C-termianl long stem domain segment of Influenza A HA subtype H2(No Cys, Ala)
PEYGFRISKRGSSGIMKTEGTLENCETKCQTPLGAINTTLPFHNVHPLTIGECPKYVKSERLVLATGLRNVPQIESR

SEQ ID NO: 498 - protein, 76 aa, Influenza virus A
  source 1..76: note = C-termianl long stem domain segment of Influenza A HA subtype H2(No Cys, Ala - Delta 1)
EYGFRISKRGSSGIMKTEGTLENCETKCQTPLGAINTTLPFHNVHPLTIGECPKYVKSERLVLATGLRNVPQIESR

SEQ ID NO: 499 - protein, 75 aa, Influenza virus A
  source 1..75: note = C-termianl long stem domain segment of Influenza A HA subtype H2(No Cys, Ala - Delta 3)
YGFRISKRGSSGIMKTEGTLENCETKCQTPLGAINTTLPFHNVHPLTIGECPKYVKSERLVLATGLRNVPQIESR

SEQ ID NO: 500 - protein, 76 aa, Influenza virus A
  source 1..76: note = C-termianl long stem domain segment of Influenza A HA subtype H3(No Cys, Ala)
PRGYFKMRTGKSSIMSSDAPIDTCISECITPNGSIPNDKPFQNVNKITYGACPKYVKQNTLKLATGMRNVPEKQTR

SEQ ID NO: 501 - protein, 75 aa, Influenza virus A
  source 1..75: note = C-termianl long stem domain segment of Influenza A HA subtype H3(No Cys, Ala - Delta 1)
RGYFKMRTGKSSIMSSDAPIDTCISECITPNGSIPNDKPFQNVNKITYGACPKYVKQNTLKLATGMRNVPEKQTR

SEQ ID NO: 502 - protein, 74 aa, Influenza virus A
  source 1..74: note = C-termianl long stem domain segment of Influenza A HA subtype H3(No Cys, Ala - Delta 3)
GYFKMRTGKSSIMSSDAPIDTCISECITPNGSIPNDKPFQNVNKITYGACPKYVKQNTLKLATGMRNVPEKQTR

SEQ ID NO: 503 - protein, 77 aa, Influenza virus A
  source 1..77: note = C-termianl long stem domain segment of Influenza A HA subtype H4(No Cys, Ala)
PRGHYKLNNQKKSTILNTAIPIGSCVSKCHTDKGSLSTTKPFQNISRIAVGDCPRYVKQGSLKLATGMRNIPEKASR

SEQ ID NO: 504 - protein, 76 aa, Influenza virus A
  source 1..76: note = C-termianl long stem domain segment of Influenza A HA subtype H4(No Cys, Ala - Delta 1)
RGHYKLNNQKKSTILNTAIPIGSCVSKCHTDKGSLSTTKPFQNISRIAVGDCPRYVKQGSLKLATGMRNIPEKASR

SEQ ID NO: 505 - protein, 75 aa, Influenza virus A
  source 1..75: note = C-termianl long stem domain segment of Influenza A HA subtype H4(No Cys, Ala - Delta 3)
GHYKLNNQKKSTILNTAIPIGSCVSKCHTDKGSLSTTKPFQNISRIAVGDCPRYVKQGSLKLATGMRNIPEKASR

SEQ ID NO: 506 - protein, 77 aa, Influenza virus A
  source 1..77: note = C-termianl long stem domain segment of Influenza A HA subtype H5(No Cys, Ala)
PRYAYKIVKKGDSAIMKSGLAYGNCDTKCQTPVGEINSSMPFHNIHPHTIGECPKYVKSDRLVLATGLRNVPQRKKR

SEQ ID NO: 507 - protein, 76 aa, Influenza virus A
  source 1..76: note = C-termianl long stem domain segment of Influenza A HA subtype H5(No Cys, Ala - Delta 1)
RYAYKIVKKGDSAIMKSGLAYGNCDTKCQTPVGEINSSMPFHNIHPHTIGECPKYVKSDRLVLATGLRNVPQRKKR

SEQ ID NO: 508 - protein, 75 aa, Influenza virus A
  source 1..75: note = C-termianl long stem domain segment of Influenza A HA subtype H5(No Cys, Ala - Delta 3)
YAYKIVKKGDSAIMKSGLAYGNCDTKCQTPVGEINSSMPFHNIHPHTIGECPKYVKSDRLVLATGLRNVPQRKKR

SEQ ID NO: 509 - protein, 78 aa, Influenza virus A
  source 1..78: note = C-termianl long stem domain segment of Influenza A HA subtype H6(No Cys, Ala)
PWYAFRFVSTSNKGAVFKSNLPIENCDATCQTVAGVLRTNKTFQNVSPLWIGECPKYVKSESLRLATGLRNVPQIETR

SEQ ID NO: 510 - protein, 77 aa, Influenza virus A
  source 1..77: note = C-termianl long stem domain segment of Influenza A HA subtype H6(No Cys, Ala - Delta 1)
WYAFRFVSTSNKGAVFKSNLPIENCDATCQTVAGVLRTNKTFQNVSPLWIGECPKYVKSESLRLATGLRNVPQIETR

SEQ ID NO: 511 - protein, 76 aa, Influenza virus A
  source 1..76: note = C-termianl long stem domain segment of Influenza A HA subtype H6(No Cys, Ala - Delta 3)
YAFRFVSTSNKGAVFKSNLPIENCDATCQTVAGVLRTNKTFQNVSPLWIGECPKYVKSESLRLATGLRNVPQIETR

SEQ ID NO: 512 - protein, 80 aa, Influenza virus A
  source 1..80: note = C-termianl long stem domain segment of Influenza A HA subtype H7(No Cys, Ala)
PNRASFLRGKSMGIQSDVQVDANCEGECYHSGGTITSRLPFQNINSRAVGKCPRYVKQESLLLATGMKNVPEPSKKRKKR

SEQ ID NO: 513 - protein, 79 aa, Influenza virus A
  source 1..79: note = C-termianl long stem domain segment of Influenza A HA subtype H7(No Cys, Ala - Delta 1)
NRASFLRGKSMGIQSDVQVDANCEGECYHSGGTITSRLPFQNINSRAVGKCPRYVKQESLLLATGMKNVPEPSKKRKKR

SEQ ID NO: 514 - protein, 78 aa, Influenza virus A
  source 1..78: note = C-termianl long stem domain segment of Influenza A HA subtype H7(No Cys, Ala - Delta 3)
RASFLRGKSMGIQSDVQVDANCEGECYHSGGTITSRLPFQNINSRAVGKCPRYVKQESLLLATGMKNVPEPSKKRKKR

SEQ ID NO: 515 - protein, 78 aa, Influenza virus A
  source 1..78: note = C-termianl long stem domain segment of Influenza A HA subtype H8(No Cys, Ala)
PEFGYLLKGESYGRIIQNEDIPIGNCNTKCQTYAGAINSSKPFQNASRHYMGECPKYVKKASLRLAVGLRNTPSVEPR

SEQ ID NO: 516 - protein, 77 aa, Influenza virus A
  source 1..77: note = C-termianl long stem domain segment of Influenza A HA subtype H8(No Cys, Ala - Delta 1)
EFGYLLKGESYGRIIQNEDIPIGNCNTKCQTYAGAINSSKPFQNASRHYMGECPKYVKKASLRLAVGLRNTPSVEPR

SEQ ID NO: 517 - protein, 76 aa, Influenza virus A
  source 1..76: note = C-termianl long stem domain segment of Influenza A HA subtype H8(No Cys, Ala - Delta 3)
FGYLLKGESYGRIIQNEDIPIGNCNTKCQTYAGAINSSKPFQNASRHYMGECPKYVKKASLRLAVGLRNTPSVEPR

SEQ ID NO: 518 - protein, 77 aa, Influenza virus A
  source 1..77: note = C-termianl long stem domain segment of Influenza A HA subtype H9(No Cys, Ala)
PWYGHVLTGESHGRILKTDLNNGNCVVQCQTEKGGLNTTLPFHNISKYAFGNCPKYVGVKSLKLPVGLRNVPAVSSR

SEQ ID NO: 519 - protein, 76 aa, Influenza virus A
  source 1..76: note = C-termianl long stem domain segment of Influenza A HA subtype H9(No Cys, Ala - Delta 1)
WYGHVLTGESHGRILKTDLNNGNCVVQCQTEKGGLNTTLPFHNISKYAFGNCPKYVGVKSLKLPVGLRNVPAVSSR

SEQ ID NO: 520 - protein, 75 aa, Influenza virus A
  source 1..75: note = C-termianl long stem domain segment of Influenza A HA subtype H9(No Cys, Ala - Delta 3)
YGHVLTGESHGRILKTDLNNGNCVVQCQTEKGGLNTTLPFHNISKYAFGNCPKYVGVKSLKLPVGLRNVPAVSSR

SEQ ID NO: 521 - protein, 77 aa, Influenza virus A
  source 1..77: note = C-termianl long stem domain segment of Influenza A HA subtype H10(No Cys, Ala)
PSRVSKLTGRDLGIQSEALIDNSCESKCFWRGGSINTKLPFQNLSPRTVGQCPKYVNQRSLLLATGMRNVPEVVQGR

SEQ ID NO: 522 - protein, 76 aa, Influenza virus A
  source 1..76: note = C-termianl long stem domain segment of Influenza A HA subtype H10(No Cys, Ala - Delta 1)
SRVSKLTGRDLGIQSEALIDNSCESKCFWRGGSINTKLPFQNLSPRTVGQCPKYVNQRSLLLATGMRNVPEVVQGR

SEQ ID NO: 523 - protein, 75 aa, Influenza virus A
  source 1..75: note = C-termianl long stem domain segment of Influenza A HA subtype H10(No Cys, Ala - Delta 3)
RVSKLTGRDLGIQSEALIDNSCESKCFWRGGSINTKLPFQNLSPRTVGQCPKYVNQRSLLLATGMRNVPEVVQGR

SEQ ID NO: 524 - protein, 77 aa, Influenza virus A
  source 1..77: note = C-termianl long stem domain segment of Influenza A HA subtype H11(No Cys, Ala)
PRYAFEIVSVGNGKLFRSELNIESCSTKCQTEIGGINTNKSFHNVHRNTIGDCPKYVNVKSLKLATGPRNVPAIASR

SEQ ID NO: 525 - protein, 76 aa, Influenza virus A
  source 1..76: note = C-termianl long stem domain segment of Influenza A HA subtype H11(No Cys, Ala - Delta 1)
RYAFEIVSVGNGKLFRSELNIESCSTKCQTEIGGINTNKSFHNVHRNTIGDCPKYVNVKSLKLATGPRNVPAIASR

SEQ ID NO: 526 - protein, 75 aa, Influenza virus A
  source 1..75: note = C-termianl long stem domain segment of Influenza A HA subtype H11(No Cys, Ala - Delta 3)
YAFEIVSVGNGKLFRSELNIESCSTKCQTEIGGINTNKSFHNVHRNTIGDCPKYVNVKSLKLATGPRNVPAIASR

SEQ ID NO: 527 - protein, 77 aa, Influenza virus A
  source 1..77: note = C-termianl long stem domain segment of Influenza A HA subtype H12(No Cys, Ala)
PEYGHLITGKSHGRILKNNLPMGQCVTECQLNEGVMNTSKPFQNTSKHYIGKCPKYIPSGSLKLAIGLRNVPQVQDR

SEQ ID NO: 528 - protein, 76 aa, Influenza virus A
  source 1..76: note = C-termianl long stem domain segment of Influenza A HA subtype H12(No Cys, Ala - Delta 1)
EYGHLITGKSHGRILKNNLPMGQCVTECQLNEGVMNTSKPFQNTSKHYIGKCPKYIPSGSLKLAIGLRNVPQVQDR

SEQ ID NO: 529 - protein, 75 aa, Influenza virus A
  source 1..75: note = C-termianl long stem domain segment of Influenza A HA subtype H12(No Cys, Ala - Delta 3)
YGHLITGKSHGRILKNNLPMGQCVTECQLNEGVMNTSKPFQNTSKHYIGKCPKYIPSGSLKLAIGLRNVPQVQDR

SEQ ID NO: 530 - protein, 77 aa, Influenza virus A
  source 1..77: note = C-termianl long stem domain segment of Influenza A HA subtype H13(No Cys, Ala)
PRYGYIIEEYGKGRIFQSRIRMSRCNTKCQTSVGGINTNRTFQNIDKNALGDCPKYIKSGQLKLATGLRNVPAISNR

SEQ ID NO: 531 - protein, 76 aa, Influenza virus A
  source 1..76: note = C-termianl long stem domain segment of Influenza A HA subtype H13(No Cys, Ala - Delta 1)
RYGYIIEEYGKGRIFQSRIRMSRCNTKCQTSVGGINTNRTFQNIDKNALGDCPKYIKSGQLKLATGLRNVPAISNR

SEQ ID NO: 532 - protein, 75 aa, Influenza virus A
  source 1..75: note = C-termianl long stem domain segment of Influenza A HA subtype H13(No Cys, Ala - Delta 3)
YGYIIEEYGKGRIFQSRIRMSRCNTKCQTSVGGINTNRTFQNIDKNALGDCPKYIKSGQLKLATGLRNVPAISNR

SEQ ID NO: 533 - protein, 77 aa, Influenza virus A
  source 1..77: note = C-termianl long stem domain segment of Influenza A HA subtype H14(No Cys, Ala)
PRGHYKISKSTKSTVLKSDKRIGSCTSPCLTDKGSIQSDKPFQNVSRIAIGNCPKYVKQGSLMLATGMRNIPGKQAK

SEQ ID NO: 534 - protein, 76 aa, Influenza virus A
  source 1..76: note = C-termianl long stem domain segment of Influenza A HA subtype H14(No Cys, Ala - Delta 1)
RGHYKISKSTKSTVLKSDKRIGSCTSPCLTDKGSIQSDKPFQNVSRIAIGNCPKYVKQGSLMLATGMRNIPGKQAK

SEQ ID NO: 535 - protein, 75 aa, Influenza virus A
  source 1..75: note = C-termianl long stem domain segment of Influenza A HA subtype H14(No Cys, Ala - Delta 3)
GHYKISKSTKSTVLKSDKRIGSCTSPCLTDKGSIQSDKPFQNVSRIAIGNCPKYVKQGSLMLATGMRNIPGKQAK

SEQ ID NO: 536 - protein, 87 aa, Influenza virus A
  source 1..87: note = C-termianl long stem domain segment of Influenza A HA subtype H15(No Cys, Ala)
PDRATFLRSNAPSGIEYNGKSLGIQSDAQIDESCEGECFYSGGTINSPLPFQNIDSRAVGKCPRYVKQSSLPLALGMKNVPEKIRTR

SEQ ID NO: 537 - protein, 86 aa, Influenza virus A
  source 1..86: note = C-termianl long stem domain segment of Influenza A HA subtype H15(No Cys, Ala - Delta 1)
DRATFLRSNAPSGIEYNGKSLGIQSDAQIDESCEGECFYSGGTINSPLPFQNIDSRAVGKCPRYVKQSSLPLALGMKNVPEKIRTR

SEQ ID NO: 538 - protein, 85 aa, Influenza virus A
  source 1..85: note = C-termianl long stem domain segment of Influenza A HA subtype H15(No Cys, Ala - Delta 3)
RATFLRSNAPSGIEYNGKSLGIQSDAQIDESCEGECFYSGGTINSPLPFQNIDSRAVGKCPRYVKQSSLPLALGMKNVPEKIRTR

SEQ ID NO: 539 - protein, 77 aa, Influenza virus A
  source 1..77: note = C-termianl long stem domain segment of Influenza A HA subtype H16(No Cys, Ala)
PRYGYIIEKYGTGRIFQSGVRMARCNTKCQTSLGGINTNKTFQNIERNALGDCPKYIKSGQLKLATGLRNVPSIGER

SEQ ID NO: 540 - protein, 76 aa, Influenza virus A
  source 1..76: note = C-termianl long stem domain segment of Influenza A HA subtype H16(No Cys, Ala - Delta 1)
RYGYIIEKYGTGRIFQSGVRMARCNTKCQTSLGGINTNKTFQNIERNALGDCPKYIKSGQLKLATGLRNVPSIGER

SEQ ID NO: 541 - protein, 75 aa, Influenza virus A
  source 1..75: note = C-termianl long stem domain segment of Influenza A HA subtype H16(No Cys, Ala - Delta 3)
YGYIIEKYGTGRIFQSGVRMARCNTKCQTSLGGINTNKTFQNIERNALGDCPKYIKSGQLKLATGLRNVPSIGER

SEQ ID NO: 542 - protein, 16 aa, synthetic construct
  source 1..16: note = linker sequence
KLNGSGIMKTEGTLEN

SEQ ID NO: 543 - protein, 5 aa, synthetic construct
  source 1..5: note = linker sequence
NNIDT

SEQ ID NO: 544 - protein, 5 aa, synthetic construct
  source 1..5: note = sequence of influenza HA polypeptide
TGLRN

SEQ ID NO: 545 - protein, 12 aa, synthetic construct
  source 1..12: note = sequence of influenza HA polypeptide
GITNKVNSVIEK

SEQ ID NO: 546 - protein, 5 aa, synthetic construct
  source 1..5: note = linker sequence
NNIDT

SEQ ID NO: 547 - protein, 5 aa, synthetic construct
  source 1..5: note = sequence of influenza HA polypeptide
TGMRN

SEQ ID NO: 548 - protein, 12 aa, synthetic construct
  source 1..12: note = sequence of influenza HA polypeptide
QINGKLNRLIEK

SEQ ID NO: 549 - protein, 12 aa, synthetic construct
  source 1..12: note = sequence of influenza HA polypeptide
QINGKLNRVIEK

SEQ ID NO: 550 - protein, 94 aa, Influenza virus B
  source 1..94: note = HA1 N-terminal Stem Segment of Influenza B HA construct variant Cys94-Cys143
DRICTGITSSNSPHVVKTATQGEVNVTGVIPLTTTPTKSHFANLKGTQTRGKLCPNCLNCTDLDVALGRPKCMGTIPSAKASILHEVKPVTSGC

SEQ ID NO: 551 - protein, 178 aa, Influenza virus B
  source 1..178: note = HA1 N-terminal Stem Segment of Influenza B HA construct variant Cys178-Cys272
DRICTGITSSNSPHVVKTATQGEVNVTGVIPLTTTPTKSHFANLKGTQTRGKLCPNCLNCTDLDVALGRPKCMGTIPSAKASILHEVKPVTSGCFPIMHDRTKIRQLPNLLRGYENIRLSARNVTNAETAPGGPYIVGTSGSCPNVTNGNGFFATMAWAVPKNKTATNPLTVEVPYIC

SEQ ID NO: 552 - protein, 54 aa, Influenza virus B
  source 1..54: note = HA1 N-terminal Stem Segment of Influenza B HA construct variant Cys54-Cys272
DRICTGITSSNSPHVVKTATQGEVNVTGVIPLTTTPTKSHFANLKGTQTRGKLC

SEQ ID NO: 553 - protein, 200 aa, Influenza virus B
  source 1..200: note = HA1 C-terminal Stem Segment of Influenza B HA construct variant Cys94-Cys143
CPNVTNGNGFFATMAWAVPKNKTATNPLTVEVPYICTKGEDQITVWGFHSDDETQMVKLYGDSKPQKFTSSANGVTTHYVSQIGGFPNQAEDEGLPQSGRIVVDYMVQKPGKTGTIAYQRGVLLPQKVWCASGRSKVIKGSLPLIGEADCLHEKYGGLNKSKPYYTGEHAKAIGNCPIWVKTPLKLANGTKYRPPAKLLK

SEQ ID NO: 554 - protein, 71 aa, Influenza virus B
  source 1..71: note = HA1 C-terminal Stem Segment of Influenza B HA construct variant Cys178-Cys272
CASGRSKVIKGSLPLIGEADCLHEKYGGLNKSKPYYTGEHAKAIGNCPIWVKTPLKLANGTKYRPPAKLLK

SEQ ID NO: 555 - protein, 94 aa, Influenza virus B; identical to SEQ ID NO: 550
  source 1..94: note = HA1 N-terminal Stem Segment of Influenza B HA construct variant Cys94-Cys143-Cys178-Cys272

SEQ ID NO: 556 - protein, 36 aa, Influenza virus B
  source 1..36: note = HA1 intermediate Segment of Influenza B HA construct variant Cys94-Cys143-Cys178-Cys272
CPNVTNGNGFFATMAWAVPKNKTATNPLTVEVPYIC

SEQ ID NO: 557 - protein, 71 aa, Influenza virus B; identical to SEQ ID NO: 554
  source 1..71: note = HA1 C-terminal Stem Segment of Influenza B HA construct variant Cys94-Cys143-Cys178-Cys272

SEQ ID NO: 558 - protein, 585 aa, Influenza virus B
  source 1..585: note = representative sequence of influenza virus B hemagglutinin (in Fig. 2)
MKAIIVILMVVTSNADRICTGITSSNSPHVVKTATQGEVNVTGVIPLTTTPTKSHFANLKGTETRGKLCPKCLNCTDLDVALGRPKCTGKIPSARVSILHEVRPVTSGCFPIMHDRTKIRQLPNLLRGYEHIRLSTHNVINAENAPGGPYKIGTSGSCPNITNGNGFFATMAWAVPKNDKNKTATNPLTIEVPYICTEGEDQITVWGFHSDSETQMAKLYGDSKPQKFTSSANGVTTHYVSQIGGFPNQTEDGGLPQSGRIVVDYMVQKSGKTGTITYQRGILLPQKVWCASGRSKVIKGSLPLIGEADCLHEKYGGLNKSKPYYTGEHAKAIGNCPIWVKTPLKLANGTKYRPPAKLLKERGFFGAIAGFLEGGWEGMIAGWHGYTSHGAHGVAVAADLKSTQEAINKITKNLNSLSELEVKNLQRLSGAMDELHNEILELDEKVDDLRADTISSQIELAVLLSNETFDSLNITAASLNDDGLDNHTILLYYSTAASSLAVTLMIAIFVVYMVSRDNVSCSICLGIINSEDEHLLALERKLKKMLGPSAVEIGNGCFETKHKCNQTCLDRIAAGTFDAGEFSLP

SEQ ID NO: 559 - protein, 16 aa, synthetic construct
  source 1..16: note = linker sequence
KLNGSGIMKTEGTLEN

SEQ ID NO: 560 - protein, 18 aa, synthetic construct
  source 1..18: note = influenza A HA subtype H17 signal peptides
MELIVLLILLNPYTFVLG

SEQ ID NO: 561 - protein, 42 aa, synthetic construct
  source 1..42: note = influenza A HA subtype H17 N-terminal stem segment
DRICIGYQANQNNQTVNTLLEQNVPVTGAQEILETNHNGKLC

SEQ ID NO: 562 - protein, 53 aa, synthetic construct
  source 1..53: note = influenza A HA subtype H17 C-terminal stem segment
CSTKCQTPLGALNSTLPFQNVHQQTIGNCPKYVKATSLMLATGLRNNPQMEGR

SEQ ID NO: 563 - protein, 222 aa, synthetic construct
  source 1..222: note = influenza A HA subtype H17 HA2 domain
GLFGAIAGFIEGGWQGMIDGWYGYHHENQEGSGYAADKEATQKAVDAITNKVNSIIDKMNSQFESNIKEFNRLELRIQHLSDRVDDALLDIWSYNTELLVLLENERTLDFHDANVKNLFEKVKAQLKDNAIDEGNGCFLLLHKCNNSCMDDIKNGTYKYMDYREESHIEKQKIDGVKLTDYSRYYIMTLYSTIASSVVLGSLIIAAFLWGCQKGSIQCKICI

SEQ ID NO: 564 - protein, 41 aa, synthetic construct
  source 1..41: note = N-terminal stem segment of Influenza A HA subtype H17(no Cys)
DRICIGYQANQNNQTVNTLLEQNVPVTGAQEILETNHNGKL

SEQ ID NO: 565 - protein, 52 aa, synthetic construct
  source 1..52: note = C-terminal stem segment of Influenza A HA subtype H17(no Cys)
STKCQTPLGALNSTLPFQNVHQQTIGNCPKYVKATSLMLATGLRNNPQMEGR

SEQ ID NO: 566 - protein, 180 aa, synthetic construct
  source 1..180: note = influenza A HA2 domain subtype H17 stem domain
GLFGAIAGFIEGGWQGMIDGWYGYHHENQEGSGYAADKEATQKAVDAITNKVNSIIDKMNSQFESNIKEFNRLELRIQHLSDRVDDALLDIWSYNTELLVLLENERTLDFHDANVKNLFEKVKAQLKDNAIDEGNGCFLLLHKCNNSCMDDIKNGTYKYMDYREESHIEKQKIDGVKLTD

SEQ ID NO: 567 - protein, 5 aa, synthetic construct
  source 1..5: note = influenza A HA2 domain subtype H17 luminal domain
YSRYY

SEQ ID NO: 568 - protein, 27 aa, synthetic construct
  source 1..27: note = influenza A HA2 domain subtype H17 transmembrane domain
IMTLYSTIASSVVLGSLIIAAFLWGCQ

SEQ ID NO: 569 - protein, 10 aa, synthetic construct
  source 1..10: note = influenza A HA2 domain subtype H17 cytoplasmic domain
KGSIQCKICI

SEQ ID NO: 570 - protein, 18 aa, synthetic construct
  source 1..18: note = influenza A HA subtype H17 signal peptide
MELIVLLILLNPYTFVLG

SEQ ID NO: 571 - protein, 42 aa, synthetic construct; identical to SEQ ID NO: 561
  source 1..42: note = influenza A HA subtype H17 N-terminal stem segment

SEQ ID NO: 572 - protein, 25 aa, synthetic construct
  source 1..25: note = influenza A HA subtype H17 C-terminal short stem segment
CPKYVKATSLMLATGLRNNPQMEGR

SEQ ID NO: 573 - protein, 222 aa, synthetic construct; identical to SEQ ID NO: 563
  source 1..222: note = influenza A HA subtype H17 HA2 domain

SEQ ID NO: 574 - protein, 41 aa, synthetic construct; identical to SEQ ID NO: 564
  source 1..41: note = influenza A HA subtype H17 N-terminal stem segment

SEQ ID NO: 575 - protein, 24 aa, synthetic construct
  source 1..24: note = influenza A HA subtype H17 C-terminal stem segment
PKYVKATSLMLATGLRNNPQMEGR

SEQ ID NO: 576 - protein, 18 aa, synthetic construct
  source 1..18: note = influenza A HA subtype H17 signal peptide
MELIVLLILLNPYTFVLG

SEQ ID NO: 577 - protein, 90 aa, synthetic construct
  source 1..90: note = influenza A HA subtype H17 N-terminal long stem segment
DRICIGYQANQNNQTVNTLLEQNVPVTGAQEILETNHNGKLCSLNGVPPLDLQSCTLAGWLLGNPNCDSLLEAEEWSYIKINESAPDDLC

SEQ ID NO: 578 - protein, 79 aa, synthetic construct
  source 1..79: note = influenza A HA subtype H17 C-terminal long stem segment
APEYGFYYKRKEGKGGLMKSKLPISDCSTKCQTPLGALNSTLPFQNVHQQTIGNCPKYVKATSLMLATGLRNNPQMEGR

SEQ ID NO: 579 - protein, 222 aa, synthetic construct; identical to SEQ ID NO: 563
  source 1..222: note = influenza A HA subtype H17 HA2 domain

SEQ ID NO: 580 - protein, 89 aa, synthetic construct
  source 1..89: note = influenza A HA subtype H17 N-terminal long stem segment
DRICIGYQANQNNQTVNTLLEQNVPVTGAQEILETNHNGKLCSLNGVPPLDLQSCTLAGWLLGNPNCDSLLEAEEWSYIKINESAPDDL

SEQ ID NO: 581 - protein, 78 aa, synthetic construct
  source 1..78: note = influenza A HA subtype H17 C-terminal long stem segment
PEYGFYYKRKEGKGGLMKSKLPISDCSTKCQTPLGALNSTLPFQNVHQQTIGNCPKYVKATSLMLATGLRNNPQMEGR

SEQ ID NO: 582 - protein, 7 aa, synthetic construct
  VARIANT 7: note = Variant - Xaa = Gly or Ser
  source 1..7: note = a cleavage site recognized by Tobacco Etch Virus (TEV) protease
ENLYFQX